European Patent Application EP 4 379 054 A1, published June 5, 2024. Title: Peptide tags and nucleic acids encoding the same. Applicant: STAND Therapeutics Co., Ltd. The sequence listing filed with the application follows.

SEQUENCE LISTING (1043 sequences)

SEQ ID NO: 1 - protein, 242 aa, synthetic construct
  SOURCE 1..242
  REGION 1..242: NOTE = Y13-259
QVQLQQSGGGLVQPGRSLKLSCVVSGFTFSNYGMNWIRQTPGKGLEWVAYISSGSSYLYYAETVKGRFTISRDNAKNTLYLQMTSLRSEDTALYYCARHEGTGTDFFDYWGQGTTVTVSSGGGGSGGGGSGGGGSDIQLTQSPHSLSASLGETVSIECLASEGISNYLAWYQQKPGKSPQLLIYYASSLQDGVPSRFSGSGSGTQFSLKISNMQPEDEGVYYCQQAYKYPSTFGAGTKLEIK

SEQ ID NO: 2 - protein, 32 aa, synthetic construct
  SOURCE 1..32
  REGION 1..32: NOTE = Tag-1-1
AHSSSAESESTSDSDSSSDSESESSSSDSEGS

SEQ ID NO: 3 - protein, 32 aa, synthetic construct
  SOURCE 1..32
  REGION 1..32: NOTE = Tag-1-2
AHSLSAELESTIDSDCSSDWESELSSSDSEGS

SEQ ID NO: 4 - protein, 32 aa, synthetic construct
  SOURCE 1..32
  REGION 1..32: NOTE = Tag-1-3
AQSSSAESESGSDSDSSSDSESESSSSDSEGS

SEQ ID NO: 5 - protein, 50 aa, synthetic construct
  SOURCE 1..50
  REGION 1..50: NOTE = Tag-4-1
NEGYREAFDEDYEQQDEDFAEQDPDGNEAFEGEYDGPNQDEYPDEAQNFE

SEQ ID NO: 6 - protein, 52 aa, synthetic construct
  SOURCE 1..52
  REGION 1..52: NOTE = Tag-2-1
DEAGSSGAPADEAGSSGAPADEAGSSGAPADEAGSSGAPADEAGSSGAPAGS

SEQ ID NO: 7 - protein, 52 aa, synthetic construct
  SOURCE 1..52
  REGION 1..52: NOTE = Tag-2-2
DEVGISLAPTDEVGISLAPTDEVGISLAPTDEVGISLAPTDEVGISLAPTGS

SEQ ID NO: 8 - protein, 52 aa, synthetic construct
  SOURCE 1..52
  REGION 1..52: NOTE = Tag-2-3
DEVMISLWPTDEVMISLWPTDEVMISLWPTDEVMISLWPTDEVMISLWPTGS

SEQ ID NO: 9 - protein, 52 aa, synthetic construct
  SOURCE 1..52
  REGION 1..52: NOTE = Tag-3-1
DFAGSSGAPADFAGSSGAPADFAGSSGAPADFAGSSGAPADFAGSSGAPAGS

SEQ ID NO: 10 - protein, 52 aa, synthetic construct
  SOURCE 1..52
  REGION 1..52: NOTE = Tag-3-2
DTAVSSIAPLDTAVSSIAPLDTAVSSIAPLDTAVSSIAPLDTAVSSIAPLGS

SEQ ID NO: 11 - protein, 52 aa, synthetic construct
  SOURCE 1..52
  REGION 1..52: NOTE = Tag-3-3
DTWVSLIAILDTWVSLIAILDTWVSLIAILDTWVSLIAILDTWVSLIAILGS

SEQ ID NO: 12 - protein, 10 aa, synthetic construct
  SOURCE 1..10
  REGION 1..10: NOTE = Myc tag
EQKLISEEDL

SEQ ID NO: 13 - protein, 9 aa, synthetic construct
  SOURCE 1..9
  REGION 1..9: NOTE = HA tag
YPYDVPDYA

SEQ ID NO: 14 - protein, 15 aa, synthetic construct
  SOURCE 1..15
  REGION 1..15: NOTE = S-tag
KETAAAKFERQHMDS

SEQ ID NO: 15 - protein, 20 aa, synthetic construct
  SOURCE 1..20
  REGION 1..20: NOTE = Membrane-localization signal
KLNPPDESGPGCMSCKCVLS

SEQ ID NO: 16 - protein, 20 aa, synthetic construct
  SOURCE 1..20
  REGION 1..20: NOTE = extracellular scFv Tag
EFGGAPEFPKPSTPPGSSGL

SEQ ID NO: 17 - protein, 49 aa, synthetic construct
  SOURCE 1..49
  REGION 1..49: NOTE = hMst1
DYEFLKSWTVEDLQKRLLALDPMMEQEIEEIRQKYQSKRQPILDAIEAK

SEQ ID NO: 18 - protein, 49 aa, synthetic construct
  SOURCE 1..49
  REGION 1..49: NOTE = hMST2
DFDFLKNLSLEELQMRLKALDPMMEREIEELRQRYTAKRQPILDAMDAK

SEQ ID NO: 19 - protein, 49 aa, synthetic construct
  SOURCE 1..49
  REGION 1..49: NOTE = hRaf1
GEVNWDAFSMPELHNFLRILQREEEEHLRQILQKYSYSRQKIQEALHAS

SEQ ID NO: 20 - protein, 49 aa, synthetic construct
  SOURCE 1..49
  REGION 1..49: NOTE = hRaf5
GEVEWDAFSIPELQNFLTILEKEEQDKIQQVQKKYDKFRQKLEEALRES

SEQ ID NO: 21 - protein, 49 aa, synthetic construct
  SOURCE 1..49
  REGION 1..49: NOTE = hSAV1
HILKWELFQLADLDTYQGMLKLLFMKELEQIVKMYEAYRQALLTELENR

SEQ ID NO: 22 - protein, 61 aa, synthetic construct
  SOURCE 1..61
  REGION 1..61: NOTE = T7C
LEDPFQSGVMLGVASTVAASPEEASVTSTEETLTPAQEAARTRAANKARKEAELAAATAEQ

SEQ ID NO: 23 - protein, 44 aa, synthetic construct
  SOURCE 1..44
  REGION 1..44: NOTE = T7B
LEDPEEASVTSTEETLTPAQEAARTRAANKARKEAELAAATAEQ

SEQ ID NO: 24 - protein, 44 aa, synthetic construct
  SOURCE 1..44
  REGION 1..44: NOTE = T7B1
LEDPEEASVTSTEETLTPAQEAARTRPPNKARKEAELAAATAEQ

SEQ ID NO: 25 - protein, 44 aa, synthetic construct
  SOURCE 1..44
  REGION 1..44: NOTE = T7B2
LEDPEEASVTSTEETLTPAQEAARTRGGNKARKEAELAAATAEQ

SEQ ID NO: 26 - protein, 41 aa, synthetic construct
  SOURCE 1..41
  REGION 1..41: NOTE = T7B3
LEDPEEASVTSTEETLTPAQEAARTRAANKARKEAELTAEQ

SEQ ID NO: 27 - protein, 44 aa, synthetic construct
  SOURCE 1..44
  REGION 1..44: NOTE = T7B4
LEDPEEASVTSTEETLTPAQEAARTRAANKARKEAELEAETAEQ

SEQ ID NO: 28 - protein, 44 aa, synthetic construct
  SOURCE 1..44
  REGION 1..44: NOTE = T7B5
LEDPEEASVTSTEETLTPAQEAARTRAAAKARKEAELAAATAEQ

SEQ ID NO: 29 - protein, 41 aa, synthetic construct
  SOURCE 1..41
  REGION 1..41: NOTE = T7B6
LEDPEEASVTSTEETLTPAQEAARTRKARKEAELAAATAEQ

SEQ ID NO: 30 - protein, 39 aa, synthetic construct
  SOURCE 1..39
  REGION 1..39: NOTE = T7B7
LEDPEEASVTSTEETLTPAQEAARTRAANKARKEAELAA

SEQ ID NO: 31 - protein, 40 aa, synthetic construct
  SOURCE 1..40
  REGION 1..40: NOTE = T7B8
LEDPEEASVTSTEETLTPAQEAARTRAANKARKEAELAAA

SEQ ID NO: 32 - protein, 44 aa, synthetic construct
  SOURCE 1..44
  REGION 1..44: NOTE = T7B9
LEDPEEASVTSTEETLTPAQEAAETEAANKARKEAELEAETAEQ

SEQ ID NO: 33 - protein, 32 aa, synthetic construct
  SOURCE 1..32
  REGION 1..32: NOTE = T7B10
LEDPTPAQEAARTRAANKARKEAELAAATAEQ

SEQ ID NO: 34 - protein, 22 aa, synthetic construct
  SOURCE 1..22
  REGION 1..22: NOTE = T7A
LEDPAANKARKEAELAAATAEQ

SEQ ID NO: 35 - protein, 22 aa, synthetic construct
  SOURCE 1..22
  REGION 1..22: NOTE = T7A1
LEDPERNKERKEAELAAATAEQ

SEQ ID NO: 36 - protein, 22 aa, synthetic construct
  SOURCE 1..22
  REGION 1..22: NOTE = T7A2
LEDPERNKERKEAELEAATAEQ

SEQ ID NO: 37 - protein, 22 aa, synthetic construct
  SOURCE 1..22
  REGION 1..22: NOTE = T7A3
LEDPERNKERKEAELEAETAEQ

SEQ ID NO: 38 - protein, 43 aa, synthetic construct
  SOURCE 1..43
  REGION 1..43: NOTE = T3
LEDPAVWEAGKVVAKGVGTADITATTSNGLIASCKVIVNAATS

SEQ ID NO: 39 - protein, 43 aa, synthetic construct
  SOURCE 1..43
  REGION 1..43: NOTE = T3A
LEDPAVWEAGKVVAKGVGTADITATTSNGLIASSEEADNAATS

SEQ ID NO: 40 - protein, 89 aa, synthetic construct
  SOURCE 1..89
  REGION 1..89: NOTE = Zif628
ERPYACPVESCDRRFSRSDELTRHIRIHTGQKPFQCRICMRNFSRSDHLTTHIRTHTGEKPFACDICGRKFARSDERKRHTKIHLRQKD

SEQ ID NO: 41 - protein, 52 aa, synthetic construct
  SOURCE 1..52
  REGION 1..52: NOTE = HinR
GRPRAITKHEQEQISRLLEKGHPRQQLAIIFGIGVSTLYRYFPASSIKKRMN

SEQ ID NO: 42 - protein, 114 aa, synthetic construct
  SOURCE 1..114
  REGION 1..114: NOTE = TrpR
  REGION 17..18: NOTE = misc_feature - Xaa can be any naturally occurring amino acid
  REGION 35..36: NOTE = misc_feature - Xaa can be any naturally occurring amino acid
  REGION 53..54: NOTE = misc_feature - Xaa can be any naturally occurring amino acid
MAQQSPYSAAMAEQRHXXQEWLRFVDLLKNAYQNXXDLHLPLLNLMLTPDERXXEALGTRVRIVEELLRGEMSQRELKNELGAGIATITRGSNSLKAAPVELRQWLEEVLLKSD

SEQ ID NO: 43 - protein, 18 aa, synthetic construct
  SOURCE 1..18
  REGION 1..18: NOTE = NE-1
TKENPRSNQEESYDDNES

SEQ ID NO: 44 - protein, 18 aa, synthetic construct
  SOURCE 1..18
  REGION 1..18: NOTE = NE-8
TKENPRTNQEESYDDNES

SEQ ID NO: 45 - protein, 18 aa, synthetic construct
  SOURCE 1..18
  REGION 1..18: NOTE = NE-9
TKENPRSNQDESYDDNES

SEQ ID NO: 46 - protein, 18 aa, synthetic construct
  SOURCE 1..18
  REGION 1..18: NOTE = NE-10
TKENPRSNQPPSYDDNES

SEQ ID NO: 47 - protein, 12 aa, synthetic construct
  SOURCE 1..12
  REGION 1..12: NOTE = PA12-tag
GVAMPGAEDDVV

SEQ ID NO: 48 - protein, 14 aa, synthetic construct
  SOURCE 1..14
  REGION 1..14: NOTE = PA14-tag
EGGVAMPGAEDDVV

SEQ ID NO: 49 - protein, 123 aa, synthetic construct
  REGION 1..123: NOTE = FATT-tag
  SOURCE 1..123
DYKDDDDVEAEESDNVDSADAEEDDSDVWWGGADTDYADGSEDKVVEVAEEEEVAEVEEEEADDDEDDEDGDEVEEEAEEPYEEATERTTSIATTTTTTTESVEEVYPGQVGYPGQVGYPGQV

SEQ ID NO: 50 - protein, 36 aa, synthetic construct
  SOURCE 1..36
GGSAQLEKELQALEKENAQLEWELQALEKELAQGAT

SEQ ID NO: 51 - protein, 288 aa, synthetic construct
  SOURCE 1..288
GEGEGGGEGGEGEGGGEGGEGEGGGEGGEGEGGGEGGEGEGGGEGGEGEGGGEGGEGEGGGEGGEGEGGGEGGEGEGGGEGGEGEGGGEGGEGEGGGEGGEGEGGGEGGEGEGGGEGGEGEGGGEGGEGEGGGEGGEGEGGGEGGEGEGGGEGGEGEGGGEGGEGEGGGEGGEGEGGGEGGEGEGGGEGGEGEGGGEGGEGEGGGEGGEGEGGGEGGEGEGGGEGGEGEGGGEGGEGEGGGEGGEGEGGGEGGEGEGGGEGGEGEGGGEGGEGEGGGEGGEGEGGGEG

SEQ ID NO: 52 - protein, 21 aa, synthetic construct
  SOURCE 1..21
ASPAAPAPASPAAPAPSAPAA

SEQ ID NO: 53 - protein, 21 aa, synthetic construct
  SOURCE 1..21
ASAAAPAAASAAASAPSAAAA

SEQ ID NO: 54 - protein, 25 aa, synthetic construct
  SOURCE 1..25
AASPAAPSAPPAAASPAAPSAPPAA

SEQ ID NO: 55 - protein, 58 aa, synthetic construct [sequence omitted]

SEQ ID NO: 56 - protein, 58 aa, synthetic construct
  SOURCE 1..58
VDNKFNKEQQNAEYEIEHLPNLNEEQENAFIQSLEDDPSQSANLLAEAKKLNDAQAPK

SEQ ID NO: 57 - protein, 58 aa, synthetic construct
  SOURCE 1..58
VDNKFNKEEEEAEEEIEHLPNLNEEQEEAFIESLEDDPSQSANLLAEAKKLNDAQAPK

SEQ ID NO: 58 - protein, 20 aa, synthetic construct
  SOURCE 1..20
KLNPPDESGPGCMSCKCVLS

SEQ ID NO: 59 - protein, 50 aa, synthetic construct; identical to SEQ ID NO: 5
  SOURCE 1..50

SEQ ID NO: 60 - protein, 60 aa, synthetic construct
  SOURCE 1..60
NEGSYREAFDSEDYEQSQDSEDFSAEQDPDGNSEAFEGSEYSDGPNSQDEYPDEAQNFSE

SEQ ID NO: 61 - protein, 70 aa, synthetic construct
  SOURCE 1..70
NEGSYRESAFDSEDYEQSQDSSEDFSAEQDSSPDGNSSEAFEGSSEYSDGPNSQDEYPDEASSQNFSSSE

SEQ ID NO: 62 - protein, 20 aa, synthetic construct
  SOURCE 1..20
YDNPYFEPQYGFPPEEDEDE

SEQ ID NO: 63 - protein, 30 aa, synthetic construct
  SOURCE 1..30
SYDSNPSYFSEPSQYGSFPPSESEDSEDSE

SEQ ID NO: 64 - protein, 40 aa, synthetic construct
  SOURCE 1..40
SSYSDSNPSYFSEPSSQSSYGSSFPPSESEDSSESDSSSE

SEQ ID NO: 65 - protein, 60 aa, synthetic construct
  SOURCE 1..60
NEGQYREAFDQEDYEQQQDQEDFQAEQDPDGNQEAFEGQEYDGPNQQDEYQPDEAQNFQE

SEQ ID NO: 66 - protein, 70 aa, synthetic construct
  SOURCE 1..70
NEGQYREQAFDQEDYEQQQDQQEDFQAEQDQQPDGNQQEAFEGQQEYQDGPNQQDEYPDEAQQQNFQQQE

SEQ ID NO: 67 - protein, 30 aa, synthetic construct
  SOURCE 1..30
QYDQNPQYFQEPQQYGQFPPQEQEDQEDQE

SEQ ID NO: 68 - protein, 40 aa, synthetic construct
  SOURCE 1..40
QQYQDQNPQYFQEPQQQQYGQQFPQPQEQEDQQEQDQQQE

SEQ ID NO: 69 - protein, 60 aa, synthetic construct
  SOURCE 1..60
NEGNYREAFDNEDYEQNQDNEDFNAEQDPDGNNEAFEGNEYNDGPNNQDEYPDEAQNFNE

SEQ ID NO: 70 - protein, 70 aa, synthetic construct
  SOURCE 1..70
NEGNYRENAFDNEDYEQNQDNNEDFNAEQDNNPDGNNNEAFEGNNEYNDGPNNQDEYPDEANNQNFNNNE

SEQ ID NO: 71 - protein, 30 aa, synthetic construct
  SOURCE 1..30
NYDNNPNYFNEPNQYGNFPPNENEDNEDNE

SEQ ID NO: 72 - protein, 40 aa, synthetic construct
  SOURCE 1..40
NNYNDNNPNYFNEPNNQNNYGNNFPPNENEDNNENDNNNE

SEQ ID NO: 73 - protein, 60 aa, synthetic construct
  SOURCE 1..60
NEGPYREAFDPEDYEQPQDPEDFPAEQDPDGNPEAFEGPEYPDGPNPQDEYPDEAQNFPE

SEQ ID NO: 74 - protein, 70 aa, synthetic construct
  SOURCE 1..70
NEGPYREPAFDPEDYEQPQDPPEDFPAEQDPPPDGNPPEAFEGPPEYPDGPNPQDEYPDEAPPQNFPPPE

SEQ ID NO: 75 - protein, 30 aa, synthetic construct
  SOURCE 1..30
PYDPNPPYFPEPPQYGPFPPPEPEDPEDPE

SEQ ID NO: 76 - protein, 40 aa, synthetic construct
  SOURCE 1..40
PPYPDPNPPYFPEPPPQPPYGPPFPPPEPEDPPEPDPPPE

SEQ ID NO: 77 - protein, 60 aa, synthetic construct
  SOURCE 1..60
NEGFYREAFDFEDYEQFQDFEDFFAEQDPDGNFEAFEGFEYFDGPNFQDEYPDEAQNFFE

SEQ ID NO: 78 - protein, 70 aa, synthetic construct
  SOURCE 1..70
NEGFYREFAFDFEDYEQFQDFFEDFFAEQDFFPDGNFFEAFEGFFEYFDGPNFQDEYPDEAFFQNFFFFE

SEQ ID NO: 79 - protein, 30 aa, synthetic construct
  SOURCE 1..30
FYDFNPFYFFEPFQYGFFPPFEFEDFEDFE

SEQ ID NO: 80 - protein, 40 aa, synthetic construct
  SOURCE 1..40
FFYFDFNPFYFFEPFFQFFYGFFFPPFEFEDFFEFDFFFE

SEQ ID NO: 81 - protein, 60 aa, synthetic construct
  SOURCE 1..60
NEGYYREAFDYEDYEQYQDYEDFYAEQDPDGNYEAFEGYEYYDGPNYQDEYPDEAQNFYE

SEQ ID NO: 82 - protein, 70 aa, synthetic construct
  SOURCE 1..70
NEGYYREYAFDYEDYEQYQDYYEDFYAEQDYYPDGNYYEAFEGYYEYYDGPNYQDEYPDEAYYQNFYYYE

SEQ ID NO: 83 - protein, 30 aa, synthetic construct
  SOURCE 1..30
YYDYNPYYFYEPYQYGYFPPYEYEDYEDYE

SEQ ID NO: 84 - protein, 40 aa, synthetic construct
  SOURCE 1..40
YYYYDYNPYYFYEPYYQYYYGYYFPPYEYEDYYEYDYYYE

SEQ ID NO: 85 - protein, 25 aa, synthetic construct
  SOURCE 1..25
GNNQDSSDSDNEADEASDDEDNDGN

SEQ ID NO: 86 - protein, 50 aa, synthetic construct
  SOURCE 1..50
NEGNREASDEDSEQQDEDNAEQDPDGNEANEGESDGPNQDENPDEAQNSE

SEQ ID NO: 87 - protein, 50 aa, synthetic construct
  SOURCE 1..50
NEGNREANDEDNEQQDEDNAEQDPDGNEANEGENDGPNQDENPDEAQNNE

SEQ ID NO: 88 - protein, 50 aa, synthetic construct; identical to SEQ ID NO: 87
  SOURCE 1..50

SEQ ID NO: 89 - protein, 50 aa, synthetic construct
  SOURCE 1..50
NEGNREANDEDNEQQDEDNAEQDQDGNEANEGENDGQNQDENPDEAQNNE

SEQ ID NO: 90 - protein, 32 aa, synthetic construct
  SOURCE 1..32
DNNESADDNNENPEDNNKNTDDNEENPNNNEN

SEQ ID NO: 91 - protein, 32 aa, synthetic construct
  SOURCE 1..32
DNSESADDNSENPEDNSKNTDDSEENPSNSES

SEQ ID NO: 92 - protein, 32 aa, synthetic construct
  SOURCE 1..32
DSSESADDSSESPEDSSKSTDDSEESPSSSES

SEQ ID NO: 93 - protein, 32 aa, synthetic construct
  SOURCE 1..32
DNQESADDNQENPEDNQKNTDDQEENPQNQEQ

SEQ ID NO: 94 - protein, 32 aa, synthetic construct
  SOURCE 1..32
DQQESADDQQEQPEDQQKQTDDQEEQPQQQEQ

SEQ ID NO: 95 - protein, 32 aa, synthetic construct
  SOURCE 1..32
DNFESADDNFENPEDNFKNTDDFEENPFNFEF

SEQ ID NO: 96 - protein, 32 aa, synthetic construct
  SOURCE 1..32
DFFESADDFFEFPEDFFKFTDDFEEFPFFFEF

SEQ ID NO: 97 - protein, 32 aa, synthetic construct
  SOURCE 1..32
DNPESADDNPENPEDNPKNTDDPEENPPNPEP

SEQ ID NO: 98 - protein, 32 aa, synthetic construct
  SOURCE 1..32
DPPESADDPPEPPEDPPKPTDDPEEPPPPPEP

SEQ ID NO: 99 - protein, 32 aa, synthetic construct
  SOURCE 1..32
DNYESADDNYENPEDNYKNTDDYEENPYNYEY

SEQ ID NO: 100 - protein, 32 aa, synthetic construct
  SOURCE 1..32
DYYESADDYYEYPEDYYKYTDDYEEYPYYYEY

SEQ ID NO: 101 - protein, 20 aa, synthetic construct
  SOURCE 1..20
NDNNNNENQNGNNNEEDEDE

SEQ ID NO: 102 - protein, 20 aa, synthetic construct
  SOURCE 1..20
NDNPNNEPQNGNPPEEDEDE

SEQ ID NO: 103 - protein, 50 aa, synthetic construct
  SOURCE 1..50
ENESEDNDEEEPNQNADDGDPNANPAAEQGGDSSDDEEGQENDQSRENEQ

SEQ ID NO: 104 - protein, 50 aa, synthetic construct
  SOURCE 1..50
QNENNGDDQDQEEGSEEQQGESDRSNEESDNEPAADDNAPEGAEEPDDNN

SEQ ID NO: 105 - protein, 20 aa, synthetic construct
  SOURCE 1..20
TDNNESADDNNENPEDNNKN

SEQ ID NO: 106 - protein, 20 aa, synthetic construct
  SOURCE 1..20
DNNESADDNNENPEDNNKNT

SEQ ID NO: 107 - protein, 20 aa, synthetic construct
  SOURCE 1..20
NNESADDNNENPEDNNKNTD

SEQ ID NO: 108 - protein, 20 aa, synthetic construct
  SOURCE 1..20
NESADDNNENPEDNNKNTDD

SEQ ID NO: 109 - protein, 20 aa, synthetic construct
  SOURCE 1..20
ESADDNNENPEDNNKNTDDN

SEQ ID NO: 110 - protein, 20 aa, synthetic construct
  SOURCE 1..20
SADDNNENPEDNNKNTDDNE

SEQ ID NO: 111 - protein, 20 aa, synthetic construct
  SOURCE 1..20
DNNENPEDNNKNTDDNEENP

SEQ ID NO: 112 - protein, 20 aa, synthetic construct
  SOURCE 1..20
NNENPEDNNKNTDDNEENPN

SEQ ID NO: 113 - protein, 20 aa, synthetic construct
  SOURCE 1..20
NENPEDNNKNTDDNEENPNN

SEQ ID NO: 114 - protein, 20 aa, synthetic construct
  SOURCE 1..20
ENPEDNNKNTDDNEENPNNN

SEQ ID NO: 115 - protein, 20 aa, synthetic construct
  SOURCE 1..20
NPEDNNKNTDDNEENPNNNE

SEQ ID NO: 116 - protein, 20 aa, synthetic construct
  SOURCE 1..20
PEDNNKNTDDNEENPNNNEN

SEQ ID NO: 117 - protein, 21 aa, synthetic construct
  SOURCE 1..21
DNNESADDNNENPEDNNKNTD

SEQ ID NO: 118 - protein, 21 aa, synthetic construct
  SOURCE 1..21
NNESADDNNENPEDNNKNTDD

SEQ ID NO: 119 - protein, 21 aa, synthetic construct
  SOURCE 1..21
NESADDNNENPEDNNKNTDDN

SEQ ID NO: 120 - protein, 21 aa, synthetic construct
  SOURCE 1..21
ESADDNNENPEDNNKNTDDNE

SEQ ID NO: 121 - protein, 21 aa, synthetic construct
  SOURCE 1..21
SADDNNENPEDNNKNTDDNEE

SEQ ID NO: 122 - protein, 21 aa, synthetic construct
  SOURCE 1..21
ADDNNENPEDNNKNTDDNEEN

SEQ ID NO: 123 - protein, 21 aa, synthetic construct
  SOURCE 1..21
DDNNENPEDNNKNTDDNEENP

SEQ ID NO: 124 - protein, 21 aa, synthetic construct
  SOURCE 1..21
DNNENPEDNNKNTDDNEENPN

SEQ ID NO: 125 - protein, 21 aa, synthetic construct
  SOURCE 1..21
NNENPEDNNKNTDDNEENPNN

SEQ ID NO: 126 - protein, 21 aa, synthetic construct
  SOURCE 1..21
NENPEDNNKNTDDNEENPNNN

SEQ ID NO: 127 - protein, 21 aa, synthetic construct
  SOURCE 1..21
ENPEDNNKNTDDNEENPNNNE

SEQ ID NO: 128 - protein, 21 aa, synthetic construct
  SOURCE 1..21
NPEDNNKNTDDNEENPNNNEN

SEQ ID NO: 129 - protein, 22 aa, synthetic construct
  SOURCE 1..22
DNNESADDNNENPEDNNKNTDD

SEQ ID NO: 130 - protein, 22 aa, synthetic construct
  SOURCE 1..22
NNESADDNNENPEDNNKNTDDN

SEQ ID NO: 131 - protein, 22 aa, synthetic construct
  SOURCE 1..22
NESADDNNENPEDNNKNTDDNE

SEQ ID NO: 132 - protein, 22 aa, synthetic construct
  SOURCE 1..22
SADDNNENPEDNNKNTDDNEEN

SEQ ID NO: 133 - protein, 22 aa, synthetic construct
  SOURCE 1..22
ADDNNENPEDNNKNTDDNEENP

SEQ ID NO: 134 - protein, 22 aa, synthetic construct
  SOURCE 1..22
DDNNENPEDNNKNTDDNEENPN

SEQ ID NO: 135 - protein, 22 aa, synthetic construct
  SOURCE 1..22
DNNENPEDNNKNTDDNEENPNN

SEQ ID NO: 136 - protein, 22 aa, synthetic construct
  SOURCE 1..22
NNENPEDNNKNTDDNEENPNNN

SEQ ID NO: 137 - protein, 22 aa, synthetic construct
  SOURCE 1..22
NENPEDNNKNTDDNEENPNNNE

SEQ ID NO: 138 - protein, 22 aa, synthetic construct
  SOURCE 1..22
ENPEDNNKNTDDNEENPNNNEN

SEQ ID NO: 139 - protein, 23 aa, synthetic construct
  SOURCE 1..23
DNNESADDNNENPEDNNKNTDDN

SEQ ID NO: 140 - protein, 23 aa, synthetic construct
  SOURCE 1..23
NNESADDNNENPEDNNKNTDDNE

SEQ ID NO: 141 - protein, 23 aa, synthetic construct
  SOURCE 1..23
NESADDNNENPEDNNKNTDDNEE

SEQ ID NO: 142 - protein, 23 aa, synthetic construct
  SOURCE 1..23
ESADDNNENPEDNNKNTDDNEEN

SEQ ID NO: 143 - protein, 23 aa, synthetic construct
  SOURCE 1..23
SADDNNENPEDNNKNTDDNEENP

SEQ ID NO: 144 - protein, 23 aa, synthetic construct
  SOURCE 1..23
ADDNNENPEDNNKNTDDNEENPN

SEQ ID NO: 145 - protein, 23 aa, synthetic construct
  SOURCE 1..23
DDNNENPEDNNKNTDDNEENPNN

SEQ ID NO: 146 - protein, 23 aa, synthetic construct
  SOURCE 1..23
DNNENPEDNNKNTDDNEENPNNN

SEQ ID NO: 147 - protein, 23 aa, synthetic construct
  SOURCE 1..23
NNENPEDNNKNTDDNEENPNNNE

SEQ ID NO: 148 - protein, 23 aa, synthetic construct
  SOURCE 1..23
NENPEDNNKNTDDNEENPNNNEN

SEQ ID NO: 149 - protein, 23 aa, synthetic construct
  SOURCE 1..23
HGNNQDSSDSDNEADEASDDEDN

SEQ ID NO: 150 - protein, 24 aa, synthetic construct
  SOURCE 1..24
DNNESADDNNENPEDNNKNTDDNE

SEQ ID NO: 151 - protein, 24 aa, synthetic construct
  SOURCE 1..24
NNESADDNNENPEDNNKNTDDNEE

SEQ ID NO: 152 - protein, 24 aa, synthetic construct
  SOURCE 1..24
NESADDNNENPEDNNKNTDDNEEN

SEQ ID NO: 153 - protein, 24 aa, synthetic construct
  SOURCE 1..24
ESADDNNENPEDNNKNTDDNEENP

SEQ ID NO: 154 - protein, 24 aa, synthetic construct
  SOURCE 1..24
SADDNNENPEDNNKNTDDNEENPN

SEQ ID NO: 155 - protein, 24 aa, synthetic construct
  SOURCE 1..24
ADDNNENPEDNNKNTDDNEENPNN

SEQ ID NO: 156 - protein, 24 aa, synthetic construct
  SOURCE 1..24
DDNNENPEDNNKNTDDNEENPNNN

SEQ ID NO: 157 - protein, 24 aa, synthetic construct
  SOURCE 1..24
DNNENPEDNNKNTDDNEENPNNNE

SEQ ID NO: 158 - protein, 24 aa, synthetic construct
  SOURCE 1..24
NNENPEDNNKNTDDNEENPNNNEN

SEQ ID NO: 159 - protein, 24 aa, synthetic construct
  SOURCE 1..24
SHGNNQDSSDSDNEADEASDDEDN

SEQ ID NO: 160 - protein, 25 aa, synthetic construct
  SOURCE 1..25
DNNESADDNNENPEDNNKNTDDNEE

SEQ ID NO: 161 - protein, 25 aa, synthetic construct
  SOURCE 1..25
NNESADDNNENPEDNNKNTDDNEEN

SEQ ID NO: 162 - protein, 25 aa, synthetic construct
  SOURCE 1..25
NESADDNNENPEDNNKNTDDNEENP

SEQ ID NO: 163 - protein, 25 aa, synthetic construct
  SOURCE 1..25
ESADDNNENPEDNNKNTDDNEENPN

SEQ ID NO: 164 - protein, 25 aa, synthetic construct
  SOURCE 1..25
SADDNNENPEDNNKNTDDNEENPNN

SEQ ID NO: 165 - protein, 25 aa, synthetic construct
  SOURCE 1..25
ADDNNENPEDNNKNTDDNEENPNNN

SEQ ID NO: 166 - protein, 25 aa, synthetic construct
  SOURCE 1..25
DDNNENPEDNNKNTDDNEENPNNNE

SEQ ID NO: 167 - protein, 25 aa, synthetic construct
  SOURCE 1..25
DNNENPEDNNKNTDDNEENPNNNEN

SEQ ID NO: 168 - protein, 25 aa, synthetic construct
  SOURCE 1..25
GSHGNNQDSSDSDNEADEASDDEDN

SEQ ID NO: 169 - protein, 25 aa, synthetic construct
  SOURCE 1..25
SHGNNQDSSDSDNEADEASDDEDND

SEQ ID NO: 170 - protein, 25 aa, synthetic construct
  SOURCE 1..25
HGNNQDSSDSDNEADEASDDEDNDG

SEQ ID NO: 171 - protein, 25 aa, synthetic construct
  SOURCE 1..25
GNNQDSSDSDNEADEASDDEDNDGN

SEQ ID NO: 172 - protein, 26 aa, synthetic construct
  SOURCE 1..26
DNNESADDNNENPEDNNKNTDDNEEN

SEQ ID NO: 173 - protein, 26 aa, synthetic construct
  SOURCE 1..26
NNESADDNNENPEDNNKNTDDNEENP

SEQ ID NO: 174 - protein, 26 aa, synthetic construct
  SOURCE 1..26
NESADDNNENPEDNNKNTDDNEENPN

SEQ ID NO: 175 - protein, 26 aa, synthetic construct
  SOURCE 1..26
ESADDNNENPEDNNKNTDDNEENPNN

SEQ ID NO: 176 - protein, 26 aa, synthetic construct
  SOURCE 1..26
SADDNNENPEDNNKNTDDNEENPNNN

SEQ ID NO: 177 - protein, 26 aa, synthetic construct
  SOURCE 1..26
ADDNNENPEDNNKNTDDNEENPNNNE

SEQ ID NO: 178 - protein, 26 aa, synthetic construct
  SOURCE 1..26
DDNNENPEDNNKNTDDNEENPNNNEN

SEQ ID NO: 179 - protein, 26 aa, synthetic construct
  SOURCE 1..26
WGSHGNNQDSSDSDNEADEASDDEDN

SEQ ID NO: 180 - protein, 26 aa, synthetic construct
  SOURCE 1..26
GSHGNNQDSSDSDNEADEASDDEDND

SEQ ID NO: 181 - protein, 26 aa, synthetic construct
  SOURCE 1..26
SHGNNQDSSDSDNEADEASDDEDNDG

SEQ ID NO: 182 - protein, 26 aa, synthetic construct
  SOURCE 1..26
HGNNQDSSDSDNEADEASDDEDNDGN

SEQ ID NO: 183 - protein, 27 aa, synthetic construct
  SOURCE 1..27
DNNESADDNNENPEDNNKNTDDNEENP

SEQ ID NO: 184 - protein, 27 aa, synthetic construct
  SOURCE 1..27
NNESADDNNENPEDNNKNTDDNEENPN

SEQ ID NO: 185 - protein, 27 aa, synthetic construct
  SOURCE 1..27
NESADDNNENPEDNNKNTDDNEENPNN

SEQ ID NO: 186 - protein, 27 aa, synthetic construct
  SOURCE 1..27
ESADDNNENPEDNNKNTDDNEENPNNN

SEQ ID NO: 187 - protein, 27 aa, synthetic construct
  SOURCE 1..27
SADDNNENPEDNNKNTDDNEENPNNNE

SEQ ID NO: 188 - protein, 27 aa, synthetic construct
  SOURCE 1..27
ADDNNENPEDNNKNTDDNEENPNNNEN

SEQ ID NO: 189 - protein, 27 aa, synthetic construct
  SOURCE 1..27
SHGNNQDSSDSDNEADEASDDEDNDGN

SEQ ID NO: 190 - protein, 27 aa, synthetic construct
  SOURCE 1..27
HGNNQDSSDSDNEADEASDDEDNDGNE

SEQ ID NO: 191 - protein, 28 aa, synthetic construct
  SOURCE 1..28
DNNESADDNNENPEDNNKNTDDNEENPN

SEQ ID NO: 192 - protein, 28 aa, synthetic construct
  SOURCE 1..28
NNESADDNNENPEDNNKNTDDNEENPNN

SEQ ID NO: 193 - protein, 28 aa, synthetic construct
  SOURCE 1..28
NESADDNNENPEDNNKNTDDNEENPNNN

SEQ ID NO: 194 - protein, 28 aa, synthetic construct
  SOURCE 1..28
ESADDNNENPEDNNKNTDDNEENPNNNE

SEQ ID NO: 195 - protein, 28 aa, synthetic construct
  SOURCE 1..28
SADDNNENPEDNNKNTDDNEENPNNNEN

SEQ ID NO: 196 - protein, 28 aa, synthetic construct
  SOURCE 1..28
SHGNNQDSSDSDNEADEASDDEDNDGNE

SEQ ID NO: 197 - protein, 29 aa, synthetic construct
  SOURCE 1..29
DNNESADDNNENPEDNNKNTDDNEENPNN

SEQ ID NO: 198 - protein, 29 aa, synthetic construct
  SOURCE 1..29
NNESADDNNENPEDNNKNTDDNEENPNNN

SEQ ID NO: 199 - protein, 29 aa, synthetic construct
  SOURCE 1..29
NESADDNNENPEDNNKNTDDNEENPNNNE

SEQ ID NO: 200 - protein, 29 aa, synthetic construct
  SOURCE 1..29
ESADDNNENPEDNNKNTDDNEENPNNNEN

SEQ ID NO: 201 - protein, 30 aa, synthetic construct
  SOURCE 1..30
DNNESADDNNENPEDNNKNTDDNEENPNNN

SEQ ID NO: 202 - protein, 30 aa, synthetic construct
  SOURCE 1..30
NNESADDNNENPEDNNKNTDDNEENPNNNE

SEQ ID NO: 203 - protein, 30 aa, synthetic construct
  SOURCE 1..30
NESADDNNENPEDNNKNTDDNEENPNNNEN

SEQ ID NO: 204 - protein, 31 aa, synthetic construct
  SOURCE 1..31
DNNESADDNNENPEDNNKNTDDNEENPNNNE

SEQ ID NO: 205 - protein, 31 aa, synthetic construct
  SOURCE 1..31
NNESADDNNENPEDNNKNTDDNEENPNNNEN

SEQ ID NO: 206 - protein, 31 aa, synthetic construct
  SOURCE 1..31
FWGSHGNNQDSSDSDNEADEASDDEDNDGNE

SEQ ID NO: 207 - protein, 31 aa, synthetic construct
  SOURCE 1..31
SHGNNQDSSDSDNEADEASDDEDNDGNEGDN

SEQ ID NO: 208 - protein, 32 aa, synthetic construct; identical to SEQ ID NO: 90
  SOURCE 1..32

SEQ ID NO: 209 - protein, 32 aa, synthetic construct
  SOURCE 1..32
SHGNNQDSSDSDNEADEASDDEDNDGNEGDNE

SEQ ID NO: 210 - protein, 20 aa, synthetic construct
  SOURCE 1..20
LEDNNEEPRDPQSPPDPPNE

SEQ ID NO: 211 - protein, 20 aa, synthetic construct
  SOURCE 1..20
EDNNEEPRDPQSPPDPPNEF

SEQ ID NO: 212 - protein, 20 aa, synthetic construct
  SOURCE 1..20
DNNEEPRDPQSPPDPPNEFG

SEQ ID NO: 213 - protein, 20 aa, synthetic construct
  SOURCE 1..20
EGEQQLKPNNSNAPNEDQEE

SEQ ID NO: 214 - protein, 20 aa, synthetic construct
  SOURCE 1..20
GEQQLKPNNSNAPNEDQEEE

SEQ ID NO: 215 - protein, 20 aa, synthetic construct
  SOURCE 1..20
KPNNSNAPNEDQEEEIQQSE

SEQ ID NO: 216 - protein, 20 aa, synthetic construct
  SOURCE 1..20
PNNSNAPNEDQEEEIQQSEQ

SEQ ID NO: 217 - protein, 20 aa, synthetic construct
  SOURCE 1..20
NNSNAPNEDQEEEIQQSEQH

SEQ ID NO: 218 - protein, 21 aa, synthetic construct
  SOURCE 1..21
EGEQQLKPNNSNAPNEDQEEE

SEQ ID NO: 219 - protein, 22 aa, synthetic construct
  SOURCE 1..22
SEGEQQLKPNNSNAPNEDQEEE

SEQ ID NO: 220 - protein, 20 aa, synthetic construct
  SOURCE 1..20
EQLNFSDDDEQGSNSPKENN

SEQ ID NO: 221 - protein, 20 aa, synthetic construct
  SOURCE 1..20
LNFSDDDEQGSNSPKENNSE

SEQ ID NO: 222 - protein, 20 aa, synthetic construct
  SOURCE 1..20
NFSDDDEQGSNSPKENNSED

SEQ ID NO: 223 - protein, 20 aa, synthetic construct
  SOURCE 1..20
FSDDDEQGSNSPKENNSEDQ

SEQ ID NO: 224 - protein, 21 aa, synthetic construct
  SOURCE 1..21
LNFSDDDEQGSNSPKENNSED

SEQ ID NO: 225 - protein, 21 aa, synthetic construct
  SOURCE 1..21
NFSDDDEQGSNSPKENNSEDQ

SEQ ID NO: 226 - protein, 22 aa, synthetic construct
  SOURCE 1..22
EQLNFSDDDEQGSNSPKENNSE

SEQ ID NO: 227 - protein, 22 aa, synthetic construct
  SOURCE 1..22
QLNFSDDDEQGSNSPKENNSED

SEQ ID NO: 228 - protein, 22 aa, synthetic construct
  SOURCE 1..22
LNFSDDDEQGSNSPKENNSEDQ

SEQ ID NO: 229 - protein, 22 aa, synthetic construct
  SOURCE 1..22
NFSDDDEQGSNSPKENNSEDQG

SEQ ID NO: 230 - protein, 23 aa, synthetic construct
  SOURCE 1..23
EQLNFSDDDEQGSNSPKENNSED

SEQ ID NO: 231 - protein, 23 aa, synthetic construct
  SOURCE 1..23
QLNFSDDDEQGSNSPKENNSEDQ

SEQ ID NO: 232 - protein, 23 aa, synthetic construct
  SOURCE 1..23
LNFSDDDEQGSNSPKENNSEDQG

SEQ ID NO: 233 - protein, 23 aa, synthetic construct
  SOURCE 1..23
NFSDDDEQGSNSPKENNSEDQGS

SEQ ID NO: 234 - protein, 24 aa, synthetic construct
  SOURCE 1..24
EQLNFSDDDEQGSNSPKENNSEDQ

SEQ ID NO: 235 - protein, 25 aa, synthetic construct
  SOURCE 1..25
EQLNFSDDDEQGSNSPKENNSEDQG

SEQ ID NO: 236 - protein, 26 aa, synthetic construct
  SOURCE 1..26
EQLNFSDDDEQGSNSPKENNSEDQGS

SEQ ID NO: 237 - protein, 20 aa, synthetic construct
  SOURCE 1..20
EEKNENDENSLSSSSDSSED

SEQ ID NO: 238 - protein, 20 aa, synthetic construct
  SOURCE 1..20
NENDENSLSSSSDSSEDKDE

SEQ ID NO: 239 - protein, 21 aa, synthetic construct
  SOURCE 1..21
KETNNSNAQNPSEEEGEGQDE

SEQ ID NO: 240 - protein, 21 aa, synthetic construct
  SOURCE 1..21
ETNNSNAQNPSEEEGEGQDED

SEQ ID NO: 241 - protein, 22 aa, synthetic construct
  SOURCE 1..22
KETNNSNAQNPSEEEGEGQDED

SEQ ID NO: 242 - protein, 20 aa, synthetic construct
  SOURCE 1..20
ENANDSSDDSGEETDESFNP

SEQ ID NO: 243 - protein, 22 aa, synthetic construct
  SOURCE 1..22
DDNESNSESAENGWDSGSNFSE

SEQ ID NO: 244 - protein, 22 aa, synthetic construct
  SOURCE 1..22
DNESNSESAENGWDSGSNFSEE

SEQ ID NO: 245 - protein, 23 aa, synthetic construct
  SOURCE 1..23
SDDNESNSESAENGWDSGSNFSE

SEQ ID NO: 246 - protein, 23 aa, synthetic construct
  SOURCE 1..23
DDNESNSESAENGWDSGSNFSEE

SEQ ID NO: 247 - protein, 24 aa, synthetic construct
  SOURCE 1..24
SDDNESNSESAENGWDSGSNFSEE

SEQ ID NO: 248 - protein, 25 aa, synthetic construct
  SOURCE 1..25
SSDDNESNSESAENGWDSGSNFSEE

SEQ ID NO: 249 - protein, 20 aa, synthetic construct
  SOURCE 1..20
SEENASSGDSEENTNSDHES

SEQ ID NO: 250 - protein, 20 aa, synthetic construct
  SOURCE 1..20
EENASSGDSEENTNSDHESE

SEQ ID NO: 251 - protein, 20 aa, synthetic construct
  SOURCE 1..20
ENASSGDSEENTNSDHESEQ

SEQ ID NO: 252 - protein, 20 aa, synthetic construct
  SOURCE 1..20
DENSENNWRNEYPEEESSDG

SEQ ID NO: 253 - protein, 20 aa, synthetic construct
  SOURCE 1..20
ENSENNWRNEYPEEESSDGD

SEQ ID NO: 254 - protein, 20 aa, synthetic construct
  SOURCE 1..20
NSENNWRNEYPEEESSDGDE

SEQ ID NO: 255 - protein, 21 aa, synthetic construct
  SOURCE 1..21
DDENSENNWRNEYPEEESSDG

SEQ ID NO: 256 - protein, 21 aa, synthetic construct
  SOURCE 1..21
DENSENNWRNEYPEEESSDGD

SEQ ID NO: 257 - protein, 21 aa, synthetic construct
  SOURCE 1..21
ENSENNWRNEYPEEESSDGDE

SEQ ID NO: 258 - protein, 21 aa, synthetic construct
  SOURCE 1..21
NSENNWRNEYPEEESSDGDED

SEQ ID NO: 259 - protein, 22 aa, synthetic construct
  SOURCE 1..22
NSENNWRNEYPEEESSDGDEDS

SEQ ID NO: 260 - protein, 23 aa, synthetic construct
  SOURCE 1..23
ENSENNWRNEYPEEESSDGDEDS

SEQ ID NO: 261 - protein, 20 aa, synthetic construct
  SOURCE 1..20
EQQNEASEENNDQQSQEVPE

SEQ ID NO: 262 - protein, 20 aa, synthetic construct
  SOURCE 1..20
QQNEASEENNDQQSQEVPEK

SEQ ID NO: 263 - protein, 20 aa, synthetic construct
  SOURCE 1..20
SKMQEDEFDQGNQEQEDNSN

SEQ ID NO: 264 - protein, 20 aa, synthetic construct
  SOURCE 1..20
KMQEDEFDQGNQEQEDNSNA

SEQ ID NO: 265 - protein, 20 aa, synthetic construct
  SOURCE 1..20
MQEDEFDQGNQEQEDNSNAE

SEQ ID NO: 266 - protein, 20 aa, synthetic construct
  SOURCE 1..20
QEDEFDQGNQEQEDNSNAEM

SEQ ID NO: 267 - protein, 20 aa, synthetic construct
  SOURCE 1..20
FDQGNQEQEDNSNAEMEEEN

SEQ ID NO: 268 - protein, 21 aa, synthetic construct
  SOURCE 1..21
EFDQGNQEQEDNSNAEMEEEN

SEQ ID NO: 269 - protein, 21 aa, synthetic construct
  SOURCE 1..21
FDQGNQEQEDNSNAEMEEENA

SEQ ID NO: 270 - protein, 21 aa, synthetic construct
  SOURCE 1..21
DQGNQEQEDNSNAEMEEENAS

SEQ ID NO: 271 - protein, 21 aa, synthetic construct
  SOURCE 1..21
QGNQEQEDNSNAEMEEENASN

SEQ ID NO: 272 - protein, 22 aa, synthetic construct
  SOURCE 1..22
EFDQGNQEQEDNSNAEMEEENA

SEQ ID NO: 273 - protein, 22 aa, synthetic construct
  SOURCE 1..22
FDQGNQEQEDNSNAEMEEENAS

SEQ ID NO: 274 - protein, 22 aa, synthetic construct
  SOURCE 1..22
DQGNQEQEDNSNAEMEEENASN

SEQ ID NO: 275 - protein, 23 aa, synthetic construct
  SOURCE 1..23
DEFDQGNQEQEDNSNAEMEEENA

SEQ ID NO: 276 - protein, 23 aa, synthetic construct
  SOURCE 1..23
EFDQGNQEQEDNSNAEMEEENAS

SEQ ID NO: 277 - protein, 23 aa, synthetic construct
  SOURCE 1..23
FDQGNQEQEDNSNAEMEEENASN

SEQ ID NO: 278 - protein, 24 aa, synthetic construct
  SOURCE 1..24
DEFDQGNQEQEDNSNAEMEEENAS

SEQ ID NO: 279 - protein, 24 aa, synthetic construct
  SOURCE 1..24
EFDQGNQEQEDNSNAEMEEENASN

SEQ ID NO: 280 - protein, 25 aa, synthetic construct
  SOURCE 1..25
QEDEFDQGNQEQEDNSNAEMEEENA

SEQ ID NO: 281 - protein, 25 aa, synthetic construct
  SOURCE 1..25
EDEFDQGNQEQEDNSNAEMEEENAS

SEQ ID NO: 282 - protein, 25 aa, synthetic construct
  SOURCE 1..25
DEFDQGNQEQEDNSNAEMEEENASN

SEQ ID NO: 283 - protein, 26 aa, synthetic construct
  SOURCE 1..26
QEDEFDQGNQEQEDNSNAEMEEENAS

SEQ ID NO: 284 - protein, 26 aa, synthetic construct
  SOURCE 1..26
EDEFDQGNQEQEDNSNAEMEEENASN

SEQ ID NO: 285 - protein, 27 aa, synthetic construct
  SOURCE 1..27
QEDEFDQGNQEQEDNSNAEMEEENASN

SEQ ID NO: 286 - protein, 21 aa, synthetic construct
  SOURCE 1..21
PSENENSQSEDSVGGDNDSEN

SEQ ID NO: 287 - protein, 20 aa, synthetic construct
  SOURCE 1..20
EVEESNPSAKEDSNPNSSGE

SEQ ID NO: 288 - protein, 20 aa, synthetic construct
  SOURCE 1..20
VEESNPSAKEDSNPNSSGED

SEQ ID NO: 289 - protein, 20 aa, synthetic construct
  SOURCE 1..20
KEENSESPLNENSDESYSEE

SEQ ID NO: 290 - protein, 20 aa, synthetic construct
  SOURCE 1..20
QPGPNHEEDADSYENMDNPD

SEQ ID NO: 291 - protein, 20 aa, synthetic construct
  SOURCE 1..20
PNHEEDADSYENMDNPDGPD

SEQ ID NO: 292 - protein, 20 aa, synthetic construct
  SOURCE 1..20
NHEEDADSYENMDNPDGPDP

SEQ ID NO: 293 - protein, 20 aa, synthetic construct
  SOURCE 1..20
DDPNSSDESNGNDDANSESD

SEQ ID NO: 294 - protein, 20 aa, synthetic construct
  SOURCE 1..20
DPNSSDESNGNDDANSESDN

SEQ ID NO: 295 - protein, 20 aa, synthetic construct
  SOURCE 1..20
PNSSDESNGNDDANSESDNN

SEQ ID NO: 296 - protein, 20 aa, synthetic construct
  SOURCE 1..20
NSSDESNGNDDANSESDNNS

SEQ ID NO: 297 - protein, 20 aa, synthetic construct
  SOURCE 1..20
SSDESNGNDDANSESDNNSS

SEQ ID NO: 298 - protein, 20 aa, synthetic construct
  SOURCE 1..20
SDESNGNDDANSESDNNSSS

SEQ ID NO: 299 - protein, 20 aa, synthetic construct
  SOURCE 1..20
DESNGNDDANSESDNNSSSR

SEQ ID NO: 300 - protein, 21 aa, synthetic construct
  SOURCE 1..21
MQGDDPNSSDESNGNDDANSE

SEQ ID NO: 301 - protein, 21 aa, synthetic construct
  SOURCE 1..21
QGDDPNSSDESNGNDDANSES

SEQ ID NO: 302 - protein, 21 aa, synthetic construct
  SOURCE 1..21
GDDPNSSDESNGNDDANSESD

SEQ ID NO: 303 - protein, 21 aa, synthetic construct
  SOURCE 1..21
DDPNSSDESNGNDDANSESDN

SEQ ID NO: 304 - protein, 21 aa, synthetic construct
  SOURCE 1..21
DPNSSDESNGNDDANSESDNN

SEQ ID NO: 305 - protein, 22 aa, synthetic construct
  SOURCE 1..22
DKSMQGDDPNSSDESNGNDDAN

SEQ ID NO: 306 - protein, 22 aa, synthetic construct
  SOURCE 1..22
SMQGDDPNSSDESNGNDDANSE

SEQ ID NO: 307 - protein, 22 aa, synthetic construct
  SOURCE 1..22
MQGDDPNSSDESNGNDDANSES

SEQ ID NO: 308 - protein, 22 aa, synthetic construct
  SOURCE 1..22
QGDDPNSSDESNGNDDANSESD

SEQ ID NO: 309 - protein, 22 aa, synthetic construct
  SOURCE 1..22
GDDPNSSDESNGNDDANSESDN

SEQ ID NO: 310 - protein, 22 aa, synthetic construct
  SOURCE 1..22
DDPNSSDESNGNDDANSESDNN

SEQ ID NO: 311 - protein, 22 aa, synthetic construct
  SOURCE 1..22
DPNSSDESNGNDDANSESDNNS

SEQ ID NO: 312 - protein, 22 aa, synthetic construct
  SOURCE 1..22
DESNGNDDANSESDNNSSSRGD

SEQ ID NO: 313 - protein, 23 aa, synthetic construct
  SOURCE 1..23
DDKSMQGDDPNSSDESNGNDDAN

SEQ ID NO: 314 - protein, 23 aa, synthetic construct
  SOURCE 1..23
DKSMQGDDPNSSDESNGNDDANS

SEQ ID NO: 315 - protein, 23 aa, synthetic construct
  SOURCE 1..23
KSMQGDDPNSSDESNGNDDANSE

SEQ ID NO: 316 - protein, 23 aa, synthetic construct
  SOURCE 1..23
SMQGDDPNSSDESNGNDDANSES

SEQ ID NO: 317 - protein, 23 aa, synthetic construct
  SOURCE 1..23
MQGDDPNSSDESNGNDDANSESD

SEQ ID NO: 318 - protein, 23 aa, synthetic construct
  SOURCE 1..23
QGDDPNSSDESNGNDDANSESDN

SEQ ID NO: 319 - protein, 23 aa, synthetic construct
  SOURCE 1..23
GDDPNSSDESNGNDDANSESDNN

SEQ ID NO: 320 - protein, 23 aa, synthetic construct
  SOURCE 1..23
DDPNSSDESNGNDDANSESDNNS

SEQ ID NO: 321 - protein, 23 aa, synthetic construct
  SOURCE 1..23
DPNSSDESNGNDDANSESDNNSS

SEQ ID NO: 322 - protein, 23 aa, synthetic construct
  SOURCE 1..23
SDESNGNDDANSESDNNSSSRGD

SEQ ID NO: 323 - protein, 23 aa, synthetic construct
  SOURCE 1..23
DESNGNDDANSESDNNSSSRGDA

SEQ ID NO: 324 - protein, 23 aa, synthetic construct
  SOURCE 1..23
DDANSESDNNSSSRGDASYNSDE

SEQ ID NO: 325 - protein, 24 aa, synthetic construct
  SOURCE 1..24
FDDKSMQGDDPNSSDESNGNDDAN

SEQ ID NO: 326 - protein, 24 aa, synthetic construct
  SOURCE 1..24
DDKSMQGDDPNSSDESNGNDDANS

SEQ ID NO: 327 - protein, 24 aa, synthetic construct
  SOURCE 1..24
DKSMQGDDPNSSDESNGNDDANSE

SEQ ID NO: 328 - protein, 24 aa, synthetic construct
  SOURCE 1..24
SMQGDDPNSSDESNGNDDANSESD

SEQ ID NO: 329 - protein, 24 aa, synthetic construct
  SOURCE 1..24
MQGDDPNSSDESNGNDDANSESDN

SEQ ID NO: 330 - protein, 24 aa, synthetic construct
  SOURCE 1..24
QGDDPNSSDESNGNDDANSESDNN

SEQ ID NO: 331 - protein, 24 aa, synthetic construct
  SOURCE 1..24
GDDPNSSDESNGNDDANSESDNNS

SEQ ID NO: 332 - protein, 24 aa, synthetic construct
  SOURCE 1..24
DDPNSSDESNGNDDANSESDNNSS

SEQ ID NO: 333 - protein, 25 aa, synthetic construct
  SOURCE 1..25
DFDDKSMQGDDPNSSDESNGNDDAN

SEQ ID NO: 334 - protein, 25 aa, synthetic construct
  SOURCE 1..25
FDDKSMQGDDPNSSDESNGNDDANS

SEQ ID NO: 335 - protein, 25 aa, synthetic construct
  SOURCE 1..25
DDKSMQGDDPNSSDESNGNDDANSE

SEQ ID NO: 336 - protein, 25 aa, synthetic construct
  SOURCE 1..25
DKSMQGDDPNSSDESNGNDDANSES

SEQ ID NO: 337 - protein, 25 aa, synthetic construct
  SOURCE 1..25
KSMQGDDPNSSDESNGNDDANSESD

SEQ ID NO: 338 - protein, 25 aa, synthetic construct
  SOURCE 1..25
SMQGDDPNSSDESNGNDDANSESDN

SEQ ID NO: 339 - protein, 25 aa, synthetic construct
  SOURCE 1..25
MQGDDPNSSDESNGNDDANSESDNN

SEQ ID NO: 340 - protein, 25 aa, synthetic construct
  SOURCE 1..25
QGDDPNSSDESNGNDDANSESDNNS

SEQ ID NO: 341 - protein, 25 aa, synthetic construct
  SOURCE 1..25
GDDPNSSDESNGNDDANSESDNNSS

SEQ ID NO: 342 - protein, 25 aa, synthetic construct
  SOURCE 1..25
DDPNSSDESNGNDDANSESDNNSSS

SEQ ID NO: 343 - protein, 26 aa, synthetic construct
  SOURCE 1..26
DFDDKSMQGDDPNSSDESNGNDDANS

SEQ ID NO: 344 - protein, 26 aa, synthetic construct
  SOURCE 1..26
FDDKSMQGDDPNSSDESNGNDDANSE

SEQ ID NO: 345 - protein, 26 aa, synthetic construct
  SOURCE 1..26
DDKSMQGDDPNSSDESNGNDDANSES

SEQ ID NO: 346 - protein, 26 aa, synthetic construct
  SOURCE 1..26
DKSMQGDDPNSSDESNGNDDANSESD

SEQ ID NO: 347 - protein, 26 aa, synthetic construct
  SOURCE 1..26
KSMQGDDPNSSDESNGNDDANSESDN

SEQ ID NO: 348 - protein, 26 aa, synthetic construct
  SOURCE 1..26
SMQGDDPNSSDESNGNDDANSESDNN

SEQ ID NO: 349 - protein, 26 aa, synthetic construct
  SOURCE 1..26
MQGDDPNSSDESNGNDDANSESDNNS

SEQ ID NO: 350 - protein, 26 aa, synthetic construct
  SOURCE 1..26
QGDDPNSSDESNGNDDANSESDNNSS

SEQ ID NO: 351 - protein, 26 aa, synthetic construct
  SOURCE 1..26
GDDPNSSDESNGNDDANSESDNNSSS

SEQ ID NO: 352 - protein, 26 aa, synthetic construct
  SOURCE 1..26
DDPNSSDESNGNDDANSESDNNSSSR

SEQ ID NO: 353 - protein, 27 aa, synthetic construct
  SOURCE 1..27
DKSMQGDDPNSSDESNGNDDANSESDN

SEQ ID NO: 354 - protein, 28 aa, synthetic construct
  SOURCE 1..28
DDKSMQGDDPNSSDESNGNDDANSESDN

SEQ ID NO: 355 - protein, 28 aa, synthetic construct
  SOURCE 1..28
DKSMQGDDPNSSDESNGNDDANSESDNN

SEQ ID NO: 356 - protein, 28 aa, synthetic construct
  SOURCE 1..28
DDPNSSDESNGNDDANSESDNNSSSRGD

SEQ ID NO: 357 - protein, 29 aa, synthetic construct
  SOURCE 1..29
FDDKSMQGDDPNSSDESNGNDDANSESDN

SEQ ID NO: 358 - protein, 29 aa, synthetic construct
  SOURCE 1..29
DDKSMQGDDPNSSDESNGNDDANSESDNN

SEQ ID NO: 359 - protein, 29 aa, synthetic construct
  SOURCE 1..29
DKSMQGDDPNSSDESNGNDDANSESDNNS

SEQ ID NO: 360 - protein, 29 aa, synthetic construct
  SOURCE 1..29
DDPNSSDESNGNDDANSESDNNSSSRGDA

SEQ ID NO: 361 - protein, 29 aa, synthetic construct
  SOURCE 1..29
DESNGNDDANSESDNNSSSRGDASYNSDE

SEQ ID NO: 362 - protein, 30 aa, synthetic construct
  SOURCE 1..30
DFDDKSMQGDDPNSSDESNGNDDANSESDN

SEQ ID NO: 363 - protein, 30 aa, synthetic construct
  SOURCE 1..30
FDDKSMQGDDPNSSDESNGNDDANSESDNN

SEQ ID NO: 364 - protein, 30 aa, synthetic construct
  SOURCE 1..30
DDKSMQGDDPNSSDESNGNDDANSESDNNS

SEQ ID NO: 365 - protein, 30 aa, synthetic construct
  SOURCE 1..30
DKSMQGDDPNSSDESNGNDDANSESDNNSS

SEQ ID NO: 366 - protein, 30 aa, synthetic construct
  SOURCE 1..30
DDPNSSDESNGNDDANSESDNNSSSRGDAS

SEQ ID NO: 367 - protein, 30 aa, synthetic construct
  SOURCE 1..30
SDESNGNDDANSESDNNSSSRGDASYNSDE

SEQ ID NO: 368 - protein, 30 aa, synthetic construct
  SOURCE 1..30
DESNGNDDANSESDNNSSSRGDASYNSDES

SEQ ID NO: 369 - protein, 31 aa, synthetic construct
  SOURCE 1..31
DFDDKSMQGDDPNSSDESNGNDDANSESDNN

SEQ ID NO: 370 - protein, 31 aa, synthetic construct
  SOURCE 1..31
FDDKSMQGDDPNSSDESNGNDDANSESDNNS

SEQ ID NO: 371 - protein, 31 aa, synthetic construct
  SOURCE 1..31
DDKSMQGDDPNSSDESNGNDDANSESDNNSS

SEQ ID NO: 372 - protein, 32 aa, synthetic construct
  SOURCE 1..32
DFDDKSMQGDDPNSSDESNGNDDANSESDNNS

SEQ ID NO: 373 - protein, 32 aa, synthetic construct
  SOURCE 1..32
FDDKSMQGDDPNSSDESNGNDDANSESDNNSS

SEQ ID NO: 374 - protein, 32 aa, synthetic construct
  SOURCE 1..32
DDKSMQGDDPNSSDESNGNDDANSESDNNSSS

SEQ ID NO: 375 - protein, 33 aa, synthetic construct
  SOURCE 1..33
DFDDKSMQGDDPNSSDESNGNDDANSESDNNSS

SEQ ID NO: 376 - protein, 33 aa, synthetic construct
  SOURCE 1..33
FDDKSMQGDDPNSSDESNGNDDANSESDNNSSS

SEQ ID NO: 377 - protein, 34 aa, synthetic construct
  SOURCE 1..34
DFDDKSMQGDDPNSSDESNGNDDANSESDNNSSS

SEQ ID NO: 378 - protein, 35 aa, synthetic construct
  SOURCE 1..35
DDPNSSDESNGNDDANSESDNNSSSRGDASYNSDE

SEQ ID NO: 379 - protein, 36 aa, synthetic construct
  SOURCE 1..36
GDDPNSSDESNGNDDANSESDNNSSSRGDASYNSDE

SEQ ID NO: 380 - protein, 36 aa, synthetic construct
  SOURCE 1..36
DDPNSSDESNGNDDANSESDNNSSSRGDASYNSDES

SEQ ID NO: 381 - protein, 40 aa, synthetic construct
  SOURCE 1..40
DSYDFDDKSMQGDDPNSSDESNGNDDANSESDNNSSSRGD

SEQ ID NO: 382 - protein, 40 aa, synthetic construct
  SOURCE 1..40
SYDFDDKSMQGDDPNSSDESNGNDDANSESDNNSSSRGDA

SEQ ID NO: 383 - protein, 40 aa, synthetic construct
  SOURCE 1..40
YDFDDKSMQGDDPNSSDESNGNDDANSESDNNSSSRGDAS

SEQ ID NO: 384 - protein, 40 aa, synthetic construct
  SOURCE 1..40
DFDDKSMQGDDPNSSDESNGNDDANSESDNNSSSRGDASY

SEQ ID NO: 385 - protein, 40 aa, synthetic construct
  SOURCE 1..40
QGDDPNSSDESNGNDDANSESDNNSSSRGDASYNSDESKD

SEQ ID NO: 386 - protein, 40 aa, synthetic construct
  SOURCE 1..40
GDDPNSSDESNGNDDANSESDNNSSSRGDASYNSDESKDN

SEQ ID NO: 387 - protein, 40 aa, synthetic construct
  SOURCE 1..40
DDPNSSDESNGNDDANSESDNNSSSRGDASYNSDESKDNG

SEQ ID NO: 388 - protein, 42 aa, synthetic construct
  SOURCE 1..42
DDKSMQGDDPNSSDESNGNDDANSESDNNSSSRGDASYNSDE

SEQ ID NO: 389 - protein, 43 aa, synthetic construct
  SOURCE 1..43
DFDDKSMQGDDPNSSDESNGNDDANSESDNNSSSRGDASYNSD

SEQ ID NO: 390 - protein, 43 aa, synthetic construct
  SOURCE 1..43
FDDKSMQGDDPNSSDESNGNDDANSESDNNSSSRGDASYNSDE

SEQ ID NO: 391 - protein, 43 aa, synthetic construct
  SOURCE 1..43
DDKSMQGDDPNSSDESNGNDDANSESDNNSSSRGDASYNSDES

SEQ ID NO: 392 - protein, 44 aa, synthetic construct
  SOURCE 1..44
DFDDKSMQGDDPNSSDESNGNDDANSESDNNSSSRGDASYNSDE

SEQ ID NO: 393 - protein, 45 aa, synthetic construct
  SOURCE 1..45
DFDDKSMQGDDPNSSDESNGNDDANSESDNNSSSRGDASYNSDES

SEQ ID NO: 394 - protein, 60 aa, synthetic construct
  SOURCE 1..60
DDPNSSDESNGNDDANSESDNNSSSRGDASYNSDESKDNGNGSDSKGAEDDDSDSTSDTN

SEQ ID NO: 395 - protein, 60 aa, synthetic construct
  SOURCE 1..60
DPNSSDESNGNDDANSESDNNSSSRGDASYNSDESKDNGNGSDSKGAEDDDSDSTSDTNN

SEQ ID NO: 396 - protein, 60 aa, synthetic construct
  SOURCE 1..60
NSSDESNGNDDANSESDNNSSSRGDASYNSDESKDNGNGSDSKGAEDDDSDSTSDTNNSD

SEQ ID NO: 397 - protein, 60 aa, synthetic construct
  SOURCE 1..60
SSDESNGNDDANSESDNNSSSRGDASYNSDESKDNGNGSDSKGAEDDDSDSTSDTNNSDS

SEQ ID NO: 398 - protein, 60 aa, synthetic construct
  SOURCE 1..60
SDESNGNDDANSESDNNSSSRGDASYNSDESKDNGNGSDSKGAEDDDSDSTSDTNNSDSN

SEQ ID NO: 399 - protein, 60 aa, synthetic construct
  SOURCE 1..60
AEDDDSDSTSDTNNSDSNGNGNNGNDDNDKSDSGKGKSDSSDSDSSDSSNSSDSSDSSDS

SEQ ID NO: 400 - protein, 60 aa, synthetic construct
  SOURCE 1..60
EDDDSDSTSDTNNSDSNGNGNNGNDDNDKSDSGKGKSDSSDSDSSDSSNSSDSSDSSDSD

SEQ ID NO: 401 - protein, 60 aa, synthetic construct
  SOURCE 1..60
DDDSDSTSDTNNSDSNGNGNNGNDDNDKSDSGKGKSDSSDSDSSDSSNSSDSSDSSDSDS

SEQ ID NO: 402 - protein, 61 aa, synthetic construct
  SOURCE 1..61
GDDPNSSDESNGNDDANSESDNNSSSRGDASYNSDESKDNGNGSDSKGAEDDDSDSTSDTN

SEQ ID NO: 403 - protein, 61 aa, synthetic construct
  SOURCE 1..61
DDPNSSDESNGNDDANSESDNNSSSRGDASYNSDESKDNGNGSDSKGAEDDDSDSTSDTNN

SEQ ID NO: 404 - protein, 62 aa, synthetic construct
  SOURCE 1..62
QGDDPNSSDESNGNDDANSESDNNSSSRGDASYNSDESKDNGNGSDSKGAEDDDSDSTSDTN

SEQ ID NO: 405 - protein, 62 aa, synthetic construct
  SOURCE 1..62
GDDPNSSDESNGNDDANSESDNNSSSRGDASYNSDESKDNGNGSDSKGAEDDDSDSTSDTNN

SEQ ID NO: 406 - protein, 62 aa, synthetic construct
  SOURCE 1..62
DDPNSSDESNGNDDANSESDNNSSSRGDASYNSDESKDNGNGSDSKGAEDDDSDSTSDTNNS

SEQ ID NO: 407 - protein, 62 aa, synthetic construct
  SOURCE 1..62
DPNSSDESNGNDDANSESDNNSSSRGDASYNSDESKDNGNGSDSKGAEDDDSDSTSDTNNSD

SEQ ID NO: 408 - protein, 63 aa, synthetic construct
  SOURCE 1..63
MQGDDPNSSDESNGNDDANSESDNNSSSRGDASYNSDESKDNGNGSDSKGAEDDDSDSTSDTN

SEQ ID NO: 409 - protein, 63 aa, synthetic construct
  SOURCE 1..63
QGDDPNSSDESNGNDDANSESDNNSSSRGDASYNSDESKDNGNGSDSKGAEDDDSDSTSDTNN

SEQ ID NO: 410 - protein, 63 aa, synthetic construct
  SOURCE 1..63
GDDPNSSDESNGNDDANSESDNNSSSRGDASYNSDESKDNGNGSDSKGAEDDDSDSTSDTNNS

SEQ ID NO: 411 - protein, 63 aa, synthetic construct
  SOURCE 1..63
DDPNSSDESNGNDDANSESDNNSSSRGDASYNSDESKDNGNGSDSKGAEDDDSDSTSDTNNSD

SEQ ID NO: 412 - protein, 63 aa, synthetic construct
  SOURCE 1..63
DPNSSDESNGNDDANSESDNNSSSRGDASYNSDESKDNGNGSDSKGAEDDDSDSTSDTNNSDS

SEQ ID NO: 413 - protein, 64 aa, synthetic construct
  SOURCE 1..64
GDDPNSSDESNGNDDANSESDNNSSSRGDASYNSDESKDNGNGSDSKGAEDDDSDSTSDTNNSD

SEQ ID NO: 414 - protein, 64 aa, synthetic construct
  SOURCE 1..64
DDPNSSDESNGNDDANSESDNNSSSRGDASYNSDESKDNGNGSDSKGAEDDDSDSTSDTNNSDS

SEQ ID NO: 415 - protein, 65 aa, synthetic construct
  SOURCE 1..65
QGDDPNSSDESNGNDDANSESDNNSSSRGDASYNSDESKDNGNGSDSKGAEDDDSDSTSDTNNSD

SEQ ID NO: 416 - protein, 65 aa, synthetic construct
  SOURCE 1..65
GDDPNSSDESNGNDDANSESDNNSSSRGDASYNSDESKDNGNGSDSKGAEDDDSDSTSDTNNSDS

SEQ ID NO: 417 - protein, 65 aa, synthetic construct
  SOURCE 1..65
DDPNSSDESNGNDDANSESDNNSSSRGDASYNSDESKDNGNGSDSKGAEDDDSDSTSDTNNSDSN

SEQ ID NO: 418 - protein, 65 aa, synthetic construct
  SOURCE 1..65
EDDDSDSTSDTNNSDSNGNGNNGNDDNDKSDSGKGKSDSSDSDSSDSSNSSDSSDSSDSDSSDSN

SEQ ID NO: 419 - protein, 66 aa, synthetic construct
  SOURCE 1..66
MQGDDPNSSDESNGNDDANSESDNNSSSRGDASYNSDESKDNGNGSDSKGAEDDDSDSTSDTNNSD

SEQ ID NO: 420 - protein, 66 aa, synthetic construct
  SOURCE 1..66
QGDDPNSSDESNGNDDANSESDNNSSSRGDASYNSDESKDNGNGSDSKGAEDDDSDSTSDTNNSDS

SEQ ID NO: 421 - protein, 66 aa, synthetic construct
  SOURCE 1..66
GDDPNSSDESNGNDDANSESDNNSSSRGDASYNSDESKDNGNGSDSKGAEDDDSDSTSDTNNSDSN

SEQ ID NO: 422 - protein, 66 aa, synthetic construct
  SOURCE 1..66
DDPNSSDESNGNDDANSESDNNSSSRGDASYNSDESKDNGNGSDSKGAEDDDSDSTSDTNNSDSNG

SEQ ID NO: 423 - protein, 66 aa, synthetic construct
  SOURCE 1..66
AEDDDSDSTSDTNNSDSNGNGNNGNDDNDKSDSGKGKSDSSDSDSSDSSNSSDSSDSSDSDSSDSN

SEQ ID NO: 424 - protein, 66 aa, synthetic construct
  SOURCE 1..66
EDDDSDSTSDTNNSDSNGNGNNGNDDNDKSDSGKGKSDSSDSDSSDSSNSSDSSDSSDSDSSDSNS

SEQ ID NO: 425 - protein, 21 aa, synthetic construct
  SOURCE 1..21
LEEDDNNENAGEDGDNDFSPS

SEQ ID NO: 426 - protein, 21 aa, synthetic construct
  SOURCE 1..21
DNNENAGEDGDNDFSPSDEEL

SEQ ID NO: 427 - protein, 21 aa, synthetic construct
  SOURCE 1..21
NNENAGEDGDNDFSPSDEELA

SEQ ID NO: 428 - protein, 21 aa, synthetic construct
  SOURCE 1..21
NENAGEDGDNDFSPSDEELAN

SEQ ID NO: 429 - protein, 22 aa, synthetic construct
  SOURCE 1..22
DNNENAGEDGDNDFSPSDEELA

SEQ ID NO: 430 - protein, 22 aa, synthetic construct
  SOURCE 1..22
NNENAGEDGDNDFSPSDEELAN

SEQ ID NO: 431 - protein, 23 aa, synthetic construct
  SOURCE 1..23
AELEEDDNNENAGEDGDNDFSPS

SEQ ID NO: 432 - protein, 23 aa, synthetic construct
  SOURCE 1..23
DDNNENAGEDGDNDFSPSDEELA

SEQ ID NO: 433 - protein, 23 aa, synthetic construct
  SOURCE 1..23
DNNENAGEDGDNDFSPSDEELAN

SEQ ID NO: 434 - protein, 24 aa, synthetic construct
  SOURCE 1..24
DDNNENAGEDGDNDFSPSDEELAN

SEQ ID NO: 435 - protein, 25 aa, synthetic construct
  SOURCE 1..25
EDDNNENAGEDGDNDFSPSDEELAN

SEQ ID NO: 436 - protein, 24 aa, synthetic construct
  SOURCE 1..24
NPADDPNNQGEDEFEEAEQVREEN

SEQ ID NO: 437 - protein, 21 aa, synthetic construct
  SOURCE 1..21
NEENTEPGAESSENADDPNKD

SEQ ID NO: 438 - protein, 21 aa, synthetic construct
  SOURCE 1..21
ENADDPNKDTSENADGQSDEN

SEQ ID NO: 439 - protein, 22 aa, synthetic construct
  SOURCE 1..22
SENADDPNKDTSENADGQSDEN

SEQ ID NO: 440 - protein, 23 aa, synthetic construct
  SOURCE 1..23
SSENADDPNKDTSENADGQSDEN

SEQ ID NO: 441 - protein, 24 aa, synthetic construct
  SOURCE 1..24
ESSENADDPNKDTSENADGQSDEN

SEQ ID NO: 442 - protein, 20 aa, synthetic construct
  SOURCE 1..20
DRDPEMENEEQPSSENDSQN

SEQ ID NO: 443 - protein, 20 aa, synthetic construct
  SOURCE 1..20
RDPEMENEEQPSSENDSQNQ

SEQ ID NO: 444 - protein, 20 aa, synthetic construct
  SOURCE 1..20
DPEMENEEQPSSENDSQNQS

SEQ ID NO: 445 - protein, 20 aa, synthetic construct
  SOURCE 1..20
PEMENEEQPSSENDSQNQSG

SEQ ID NO: 446 - protein, 20 aa, synthetic construct
  SOURCE 1..20
EMENEEQPSSENDSQNQSGE

SEQ ID NO: 447 - protein, 20 aa, synthetic construct
  SOURCE 1..20
MENEEQPSSENDSQNQSGEQ

SEQ ID NO: 448 - protein, 20 aa, synthetic construct
  SOURCE 1..20
ENEEQPSSENDSQNQSGEQI

SEQ ID NO: 449 - protein, 21 aa, synthetic construct
  SOURCE 1..21
DSESANVSDKEAGSNENDDQN

SEQ ID NO: 450 - protein, 20 aa, synthetic construct
  SOURCE 1..20
NYNDGSQEDRDWQDDQSDNQ

SEQ ID NO: 451 - protein, 20 aa, synthetic construct
  SOURCE 1..20
RENTNEASSEGNSSDDSEDE

SEQ ID NO: 452 - protein, 20 aa, synthetic construct
  SOURCE 1..20
ENTNEASSEGNSSDDSEDER

SEQ ID NO: 453 - protein, 20 aa, synthetic construct
  SOURCE 1..20
QENDNGNETESEQPKESNEN

SEQ ID NO: 454 - protein, 20 aa, synthetic construct
  SOURCE 1..20
ENDNGNETESEQPKESNENQ

SEQ ID NO: 455 - protein, 20 aa, synthetic construct
  SOURCE 1..20
NDNGNETESEQPKESNENQE

SEQ ID NO: 456 - protein, 21 aa, synthetic construct
  SOURCE 1..21
QENDNGNETESEQPKESNENQ

SEQ ID NO: 457 - protein, 21 aa, synthetic construct
  SOURCE 1..21
ENDNGNETESEQPKESNENQE

SEQ ID NO: 458 - protein, 22 aa, synthetic construct
  SOURCE 1..22
QENDNGNETESEQPKESNENQE

SEQ ID NO: 459 - protein, 20 aa, synthetic construct
  SOURCE 1..20
QNEENPGDEEAKNQVNSESD

SEQ ID NO: 460 - protein, 20 aa, synthetic construct
  SOURCE 1..20
NEENPGDEEAKNQVNSESDS

SEQ ID NO: 461 - protein, 20 aa, synthetic construct
  SOURCE 1..20
EENPGDEEAKNQVNSESDSD

SEQ ID NO: 462 - protein, 20 aa, synthetic construct
  SOURCE 1..20
ENPGDEEAKNQVNSESDSDS

SEQ ID NO: 463 - protein, 20 aa, synthetic construct
  SOURCE 1..20
NPGDEEAKNQVNSESDSDSE

SEQ ID NO: 464 - protein, 21 aa, synthetic construct
  SOURCE 1..21
QNEENPGDEEAKNQVNSESDS

SEQ ID NO: 465 - protein, 21 aa, synthetic construct
  SOURCE 1..21
NEENPGDEEAKNQVNSESDSD

SEQ ID NO: 466 - protein, 22 aa, synthetic construct
  SOURCE 1..22
QNEENPGDEEAKNQVNSESDSD

SEQ ID NO: 467 - protein, 22 aa, synthetic construct
  SOURCE 1..22
NEENPGDEEAKNQVNSESDSDS

SEQ ID NO: 468 - protein, 23 aa, synthetic construct
  SOURCE 1..23
QNEENPGDEEAKNQVNSESDSDS

SEQ ID NO: 469 - protein, 23 aa, synthetic construct
  SOURCE 1..23
NEENPGDEEAKNQVNSESDSDSE

SEQ ID NO: 470 - protein, 24 aa, synthetic construct
  SOURCE 1..24
QNEENPGDEEAKNQVNSESDSDSE

SEQ ID NO: 471 - protein, 24 aa, synthetic construct
  SOURCE 1..24
NEENPGDEEAKNQVNSESDSDSEE

SEQ ID NO: 472 - protein, 25 aa, synthetic construct
  SOURCE 1..25
QNEENPGDEEAKNQVNSESDSDSEE

SEQ ID NO: 473 - protein, 25 aa, synthetic construct
  SOURCE 1..25
NEENPGDEEAKNQVNSESDSDSEES

SEQ ID NO: 474 - protein, 26 aa, synthetic construct
  SOURCE 1..26
QNEENPGDEEAKNQVNSESDSDSEES

SEQ ID NO: 475 - protein, 21 aa, synthetic construct
  SOURCE 1..21
YNGGNANPRPANNEEEEDEED

SEQ ID NO: 476 - protein, 21 aa, synthetic construct
  SOURCE 1..21
NGGNANPRPANNEEEEDEEDE

SEQ ID NO: 477 - protein, 21 aa, synthetic construct
  SOURCE 1..21
GGNANPRPANNEEEEDEEDEY

SEQ ID NO: 478 - protein, 22 aa, synthetic construct
  SOURCE 1..22
YNGGNANPRPANNEEEEDEEDE

SEQ ID NO: 479 - protein, 22 aa, synthetic construct
  SOURCE 1..22
NGGNANPRPANNEEEEDEEDEY

SEQ ID NO: 480 - protein, 23 aa, synthetic construct
  SOURCE 1..23
NGGNANPRPANNEEEEDEEDEYD

SEQ ID NO: 481 - protein, 20 aa, synthetic construct
  SOURCE 1..20
GASENEEEDDDYNKPLDPNS

SEQ ID NO: 482 - protein, 20 aa, synthetic construct
  SOURCE 1..20
LQNQKEAEEPGPDSENSQEN

SEQ ID NO: 483 - protein, 20 aa, synthetic construct
  SOURCE 1..20
QNQKEAEEPGPDSENSQENP

SEQ ID NO: 484 - protein, 20 aa, synthetic construct
  SOURCE 1..20
NQKEAEEPGPDSENSQENPP

SEQ ID NO: 485 - protein, 21 aa, synthetic construct
  SOURCE 1..21
KESVSPENNEEGGNDNQDNEN

SEQ ID NO: 486 - protein, 21 aa, synthetic construct
  SOURCE 1..21
ESVSPENNEEGGNDNQDNENP

SEQ ID NO: 487 - protein, 22 aa, synthetic construct
  SOURCE 1..22
KESVSPENNEEGGNDNQDNENP

SEQ ID NO: 488 - protein, 20 aa, synthetic construct
  SOURCE 1..20
ASPQPREPSDDENSDNSNEC

SEQ ID NO: 489 - protein, 21 aa, synthetic construct
  SOURCE 1..21
NNSQDEDGFQELNENGNAKDE

SEQ ID NO: 490 - protein, 21 aa, synthetic construct
  SOURCE 1..21
NSQDEDGFQELNENGNAKDEN

SEQ ID NO: 491 - protein, 22 aa, synthetic construct
  SOURCE 1..22
NNSQDEDGFQELNENGNAKDEN

SEQ ID NO: 492 - protein, 20 aa, synthetic construct
  SOURCE 1..20
SSDSPKDQSPPEDSGESEAD

SEQ ID NO: 493 - protein, 20 aa, synthetic construct
  SOURCE 1..20
PGPEPEPEPEPEPEPAPEPE

SEQ ID NO: 494 - protein, 20 aa, synthetic construct
  SOURCE 1..20
GPEPEPEPEPEPEPAPEPEP

SEQ ID NO: 495 - protein, 20 aa, synthetic construct
  SOURCE 1..20
PEPEPEPEPEPAPEPEPEPK

SEQ ID NO: 496 - protein, 20 aa, synthetic construct
  SOURCE 1..20
EPEPEPEPEPAPEPEPEPKP

SEQ ID NO: 497 - protein, 20 aa, synthetic construct
  SOURCE 1..20
PEPEPEPEPAPEPEPEPKPG

SEQ ID NO: 498 - protein, 21 aa, synthetic construct
  SOURCE 1..21
AGPGPEPEPEPEPEPEPAPEP

SEQ ID NO: 499 - protein, 21 aa, synthetic construct
  SOURCE 1..21
GPGPEPEPEPEPEPEPAPEPE

SEQ ID NO: 500 - protein, 21 aa, synthetic construct
  SOURCE 1..21
PGPEPEPEPEPEPEPAPEPEP

SEQ ID NO: 501 - protein, 21 aa, synthetic construct
  SOURCE 1..21
GPEPEPEPEPEPEPAPEPEPE

SEQ ID NO: 502 - protein, 21 aa, synthetic construct
  SOURCE 1..21
PEPEPEPEPEPEPAPEPEPEP

SEQ ID NO: 503 - protein, 21 aa, synthetic construct
  SOURCE 1..21
EPEPEPEPEPEPAPEPEPEPK

SEQ ID NO: 504 - protein, 21 aa, synthetic construct
  SOURCE 1..21
PEPEPEPEPEPAPEPEPEPKP

SEQ ID NO: 505 - protein, 21 aa, synthetic construct
  SOURCE 1..21
EPEPEPEPEPAPEPEPEPKPG

SEQ ID NO: 506 - protein, 21 aa, synthetic construct
  SOURCE 1..21
PEPEPEPEPAPEPEPEPKPGA

SEQ ID NO: 507 - protein, 21 aa, synthetic construct
  SOURCE 1..21
EPEPEPEPAPEPEPEPKPGAG

SEQ ID NO: 508 - protein, 22 aa, synthetic construct
  SOURCE 1..22
AGPGPEPEPEPEPEPEPAPEPE

SEQ ID NO: 509 - protein, 22 aa, synthetic construct
  SOURCE 1..22
GPGPEPEPEPEPEPEPAPEPEP

SEQ ID NO: 510 - protein, 22 aa, synthetic construct
  SOURCE 1..22
PGPEPEPEPEPEPEPAPEPEPE

SEQ ID NO: 511 - protein, 22 aa, synthetic construct
  SOURCE 1..22
GPEPEPEPEPEPEPAPEPEPEP

SEQ ID NO: 512 - protein, 22 aa, synthetic construct
  SOURCE 1..22
PEPEPEPEPEPEPAPEPEPEPK

SEQ ID NO: 513 - protein, 22 aa, synthetic construct
  SOURCE 1..22
EPEPEPEPEPEPAPEPEPEPKP

SEQ ID NO: 514 - protein, 22 aa, synthetic construct
  SOURCE 1..22
PEPEPEPEPEPAPEPEPEPKPG

SEQ ID NO: 515 - protein, 22 aa, synthetic construct
  SOURCE 1..22
EPEPEPEPEPAPEPEPEPKPGA

SEQ ID NO: 516 - protein, 22 aa, synthetic construct
  SOURCE 1..22
PEPEPEPEPAPEPEPEPKPGAG

SEQ ID NO: 517 - protein, 23 aa, synthetic construct
  SOURCE 1..23
AGPGPEPEPEPEPEPEPAPEPEP

SEQ ID NO: 518 - protein, 23 aa, synthetic construct
  SOURCE 1..23
GPGPEPEPEPEPEPEPAPEPEPE

SEQ ID NO: 519 - protein, 23 aa, synthetic construct
  SOURCE 1..23
PGPEPEPEPEPEPEPAPEPEPEP

SEQ ID NO: 520 - protein, 23 aa, synthetic construct
  SOURCE 1..23
GPEPEPEPEPEPEPAPEPEPEPK

SEQ ID NO: 521 - protein, 23 aa, synthetic construct
  SOURCE 1..23
PEPEPEPEPEPEPAPEPEPEPKP

SEQ ID NO: 522 - protein, 23 aa, synthetic construct
  SOURCE 1..23
EPEPEPEPEPEPAPEPEPEPKPG

SEQ ID NO: 523 - protein, 23 aa, synthetic construct
  SOURCE 1..23
PEPEPEPEPEPAPEPEPEPKPGA

SEQ ID NO: 524 - protein, 23 aa, synthetic construct
  SOURCE 1..23
EPEPEPEPEPAPEPEPEPKPGAG

SEQ ID NO: 525 - protein, 24 aa, synthetic construct
  SOURCE 1..24
AGPGPEPEPEPEPEPEPAPEPEPE

SEQ ID NO: 526 - protein, 24 aa, synthetic construct
  SOURCE 1..24
GPGPEPEPEPEPEPEPAPEPEPEP

SEQ ID NO: 527 - protein, 24 aa, synthetic construct
  SOURCE 1..24
PGPEPEPEPEPEPEPAPEPEPEPK

SEQ ID NO: 528 - protein, 24 aa, synthetic construct
  SOURCE 1..24
GPEPEPEPEPEPEPAPEPEPEPKP

SEQ ID NO: 529 - protein, 24 aa, synthetic construct
  SOURCE 1..24
PEPEPEPEPEPEPAPEPEPEPKPG

SEQ ID NO: 530 - protein, 24 aa, synthetic construct
  SOURCE 1..24
EPEPEPEPEPEPAPEPEPEPKPGA

SEQ ID NO: 531 - protein, 24 aa, synthetic construct
  SOURCE 1..24
PEPEPEPEPEPAPEPEPEPKPGAG

SEQ ID NO: 532 - protein, 25 aa, synthetic construct
  SOURCE 1..25
AGPGPEPEPEPEPEPEPAPEPEPEP

SEQ ID NO: 533 - protein, 25 aa, synthetic construct
  SOURCE 1..25
GPGPEPEPEPEPEPEPAPEPEPEPK

SEQ ID NO: 534 - protein, 25 aa, synthetic construct
  SOURCE 1..25
PGPEPEPEPEPEPEPAPEPEPEPKP

SEQ ID NO: 535 - protein, 25 aa, synthetic construct
  SOURCE 1..25
GPEPEPEPEPEPEPAPEPEPEPKPG

SEQ ID NO: 536 - protein, 25 aa, synthetic construct
  SOURCE 1..25
PEPEPEPEPEPEPAPEPEPEPKPGA

SEQ ID NO: 537 - protein, 25 aa, synthetic construct
  SOURCE 1..25
EPEPEPEPEPEPAPEPEPEPKPGAG

SEQ ID NO: 538 - protein, 26 aa, synthetic construct
  SOURCE 1..26
AGPGPEPEPEPEPEPEPAPEPEPEPK

SEQ ID NO: 539 - protein, 26 aa, synthetic construct
  SOURCE 1..26
GPGPEPEPEPEPEPEPAPEPEPEPKP

SEQ ID NO: 540 - protein, 26 aa, synthetic construct
  SOURCE 1..26
PGPEPEPEPEPEPEPAPEPEPEPKPG

SEQ ID NO: 541 - protein, 26 aa, synthetic construct
  SOURCE 1..26
GPEPEPEPEPEPEPAPEPEPEPKPGA

SEQ ID NO: 542 - protein, 26 aa, synthetic construct
  SOURCE 1..26
PEPEPEPEPEPEPAPEPEPEPKPGAG

SEQ ID NO: 543 - protein, 27 aa, synthetic construct
  SOURCE 1..27
AGPGPEPEPEPEPEPEPAPEPEPEPKP

SEQ ID NO: 544 - protein, 27 aa, synthetic construct
  SOURCE 1..27
PGPEPEPEPEPEPEPAPEPEPEPKPGA

SEQ ID NO: 545 - protein, 20 aa, synthetic construct
  SOURCE 1..20
DPEEDGSPDPEPSPEPEPKP

SEQ ID NO: 546 - protein, 20 aa, synthetic construct
  SOURCE 1..20
PEEDGSPDPEPSPEPEPKPS

SEQ ID NO: 547 - protein, 21 aa, synthetic construct
  SOURCE 1..21
EDPEEDGSPDPEPSPEPEPKP

SEQ ID NO: 548 - protein, 21 aa, synthetic construct
  SOURCE 1..21
DPEEDGSPDPEPSPEPEPKPS

SEQ ID NO: 549 - protein, 22 aa, synthetic construct
  SOURCE 1..22
EDPEEDGSPDPEPSPEPEPKPS

SEQ ID NO: 550 - protein, 23 aa, synthetic construct
  SOURCE 1..23
DEDPEEDGSPDPEPSPEPEPKPS

SEQ ID NO: 551 - protein, 21 aa, synthetic construct
  SOURCE 1..21
PDDDGSDDSSPPSASPAESEP

SEQ ID NO: 552 - protein, 21 aa, synthetic construct
  SOURCE 1..21
DDDGSDDSSPPSASPAESEPQ

SEQ ID NO: 553 - protein, 22 aa, synthetic construct
  SOURCE 1..22
PDDDGSDDSSPPSASPAESEPQ

SEQ ID NO: 554 - protein, 21 aa, synthetic construct
  SOURCE 1..21
PPPEEQGQGDAPPQHEDEEPA

SEQ ID NO: 555 - protein, 20 aa, synthetic construct
  SOURCE 1..20
PSPAPSPDSDSDSDSDGEEE

SEQ ID NO: 556 - protein, 21 aa, synthetic construct
  SOURCE 1..21
GAPSPAPSPDSDSDSDSDGEE

SEQ ID NO: 557 - protein, 21 aa, synthetic construct
  SOURCE 1..21
APSPAPSPDSDSDSDSDGEEE

SEQ ID NO: 558 - protein, 21 aa, synthetic construct
  SOURCE 1..21
PSPAPSPDSDSDSDSDGEEEE

SEQ ID NO: 559 - protein, 22 aa, synthetic construct
  SOURCE 1..22
NGAPSPAPSPDSDSDSDSDGEE

SEQ ID NO: 560 - protein, 22 aa, synthetic construct
  SOURCE 1..22
GAPSPAPSPDSDSDSDSDGEEE

SEQ ID NO: 561 - protein, 22 aa, synthetic construct
  SOURCE 1..22
APSPAPSPDSDSDSDSDGEEEE

SEQ ID NO: 562 - protein, 23 aa, synthetic construct
  SOURCE 1..23
QNGAPSPAPSPDSDSDSDSDGEE

SEQ ID NO: 563 - protein, 23 aa, synthetic construct
  SOURCE 1..23
NGAPSPAPSPDSDSDSDSDGEEE

SEQ ID NO: 564 - protein, 23 aa, synthetic construct
  SOURCE 1..23
GAPSPAPSPDSDSDSDSDGEEEE

SEQ ID NO: 565 - protein, 23 aa, synthetic construct
  SOURCE 1..23
APSPAPSPDSDSDSDSDGEEEEE

SEQ ID NO: 566 - protein, 24 aa, synthetic construct
  SOURCE 1..24
QNGAPSPAPSPDSDSDSDSDGEEE

SEQ ID NO: 567 - protein, 24 aa, synthetic construct
  SOURCE 1..24
NGAPSPAPSPDSDSDSDSDGEEEE

SEQ ID NO: 568 - protein, 24 aa, synthetic construct
  SOURCE 1..24
GAPSPAPSPDSDSDSDSDGEEEEE

SEQ ID NO: 569 - protein, 25 aa, synthetic construct
  SOURCE 1..25
QNGAPSPAPSPDSDSDSDSDGEEEE

SEQ ID NO: 570 - protein, 25 aa, synthetic construct
  SOURCE 1..25
NGAPSPAPSPDSDSDSDSDGEEEEE

SEQ ID NO: 571 - protein, 25 aa, synthetic construct
  SOURCE 1..25
GAPSPAPSPDSDSDSDSDGEEEEEE

SEQ ID NO: 572 - protein, 26 aa, synthetic construct
  SOURCE 1..26
QNGAPSPAPSPDSDSDSDSDGEEEEE

SEQ ID NO: 573 - protein, 26 aa, synthetic construct
  SOURCE 1..26
NGAPSPAPSPDSDSDSDSDGEEEEEE

SEQ ID NO: 574 - protein, 27 aa, synthetic construct
  SOURCE 1..27
QNGAPSPAPSPDSDSDSDSDGEEEEEE

SEQ ID NO: 575 - protein, 27 aa, synthetic construct
  SOURCE 1..27
NGAPSPAPSPDSDSDSDSDGEEEEEEE

SEQ ID NO: 576 - protein, 28 aa, synthetic construct
  SOURCE 1..28
QNGAPSPAPSPDSDSDSDSDGEEEEEEE

SEQ ID NO: 577 - protein, 31 aa, synthetic construct
  SOURCE 1..31
QNGAPSPAPSPDSDSDSDSDGEEEEEEEGER

SEQ ID NO: 578 - protein, 32 aa, synthetic construct
  SOURCE 1..32
QNGAPSPAPSPDSDSDSDSDGEEEEEEEGERD

SEQ ID NO: 579 - protein, 20 aa, synthetic construct
  SOURCE 1..20
EPPAPPPPPPPEEDPEQDSG

SEQ ID NO: 580 - protein, 20 aa, synthetic construct
  SOURCE 1..20
PAPPPPPPPEEDPEQDSGPE

SEQ ID NO: 581 - protein, 20 aa, synthetic construct
  SOURCE 1..20
APPPPPPPEEDPEQDSGPED

SEQ ID NO: 582 - protein, 21 aa, synthetic construct
  SOURCE 1..21
PAPPPPPPPEEDPEQDSGPED

SEQ ID NO: 583 - protein, 22 aa, synthetic construct
  SOURCE 1..22
EPPAPPPPPPPEEDPEQDSGPE

SEQ ID NO: 584 - protein, 22 aa, synthetic construct
  SOURCE 1..22
PPAPPPPPPPEEDPEQDSGPED

SEQ ID NO: 585 - protein, 23 aa, synthetic construct
  SOURCE 1..23
AEPPAPPPPPPPEEDPEQDSGPE

SEQ ID NO: 586 - protein, 23 aa, synthetic construct
  SOURCE 1..23
EPPAPPPPPPPEEDPEQDSGPED

SEQ ID NO: 587 - protein, 24 aa, synthetic construct
  SOURCE 1..24
AEPPAPPPPPPPEEDPEQDSGPED

SEQ ID NO: 588 - protein, 20 aa, synthetic construct
  SOURCE 1..20
PPPPPQAPPEEENESEPEEP

SEQ ID NO: 589 - protein, 20 aa, synthetic construct
  SOURCE 1..20
PPPPQAPPEEENESEPEEPS

SEQ ID NO: 590 - protein, 20 aa, synthetic construct
  SOURCE 1..20
PPPQAPPEEENESEPEEPSG

SEQ ID NO: 591 - protein, 21 aa, synthetic construct
  SOURCE 1..21
PPPPPQAPPEEENESEPEEPS

SEQ ID NO: 592 - protein, 21 aa, synthetic construct
  SOURCE 1..21
PPPPQAPPEEENESEPEEPSG

SEQ ID NO: 593 - protein, 22 aa, synthetic construct
  SOURCE 1..22
PPPPPQAPPEEENESEPEEPSG

SEQ ID NO: 594 - protein, 20 aa, synthetic construct
  SOURCE 1..20
PQDSSSKSPEPSADESPDND

SEQ ID NO: 595 - protein, 20 aa, synthetic construct
  SOURCE 1..20
QSSDNSEDEEEPPDNADSKS

SEQ ID NO: 596 - protein, 21 aa, synthetic construct
  SOURCE 1..21
EEEEEQPGKAPDPQDPQDAES

SEQ ID NO: 597 - protein, 21 aa, synthetic construct
  SOURCE 1..21
EEEEQPGKAPDPQDPQDAESD

SEQ ID NO: 598 - protein, 21 aa, synthetic construct
  SOURCE 1..21
EEEQPGKAPDPQDPQDAESDS

SEQ ID NO: 599 - protein, 22 aa, synthetic construct
  SOURCE 1..22
EEEEQPGKAPDPQDPQDAESDS

SEQ ID NO: 600 - protein, 23 aa, synthetic construct
  SOURCE 1..23
EEEEEQPGKAPDPQDPQDAESDS

SEQ ID NO: 601 - protein, 20 aa, synthetic construct
  SOURCE 1..20
PPPPPSEEEGPEEPPKASPE

SEQ ID NO: 602 - protein, 20 aa, synthetic construct
  SOURCE 1..20
PPPPSEEEGPEEPPKASPES

SEQ ID NO: 603 - protein, 20 aa, synthetic construct
  SOURCE 1..20
PPPSEEEGPEEPPKASPESE

SEQ ID NO: 604 - protein, 21 aa, synthetic construct
  SOURCE 1..21
PPPPSEEEGPEEPPKASPESE

SEQ ID NO: 605 - protein, 21 aa, synthetic construct
  SOURCE 1..21
PPPSEEEGPEEPPKASPESEA

SEQ ID NO: 606 - protein, 22 aa, synthetic construct
  SOURCE 1..22
PPPPPSEEEGPEEPPKASPESE

SEQ ID NO: 607 - protein, 22 aa, synthetic construct
  SOURCE 1..22
PPPPSEEEGPEEPPKASPESEA

SEQ ID NO: 608 - protein, 23 aa, synthetic construct
  SOURCE 1..23
PPPPPSEEEGPEEPPKASPESEA

SEQ ID NO: 609 - protein, 20 aa, synthetic construct
  SOURCE 1..20
DDAEEPESPPPPPRSPSPEP

SEQ ID NO: 610 - protein, 20 aa, synthetic construct
  SOURCE 1..20
SGEASSSEEEPPSPDDKENQ

SEQ ID NO: 611 - protein, 21 aa, synthetic construct
  SOURCE 1..21
SGEASSSEEEPPSPDDKENQA

SEQ ID NO: 612 - protein, 21 aa, synthetic construct
  SOURCE 1..21
GEASSSEEEPPSPDDKENQAP

SEQ ID NO: 613 - protein, 22 aa, synthetic construct
  SOURCE 1..22
SGEASSSEEEPPSPDDKENQAP

SEQ ID NO: 614 - protein, 20 aa, synthetic construct
  SOURCE 1..20
PQPPPPPPPEESSDSEPEAE

SEQ ID NO: 615 - protein, 20 aa, synthetic construct
  SOURCE 1..20
QPPPPPPPEESSDSEPEAEP

SEQ ID NO: 616 - protein, 20 aa, synthetic construct
  SOURCE 1..20
PPPPPPPEESSDSEPEAEPG

SEQ ID NO: 617 - protein, 20 aa, synthetic construct
  SOURCE 1..20
PPPPPPEESSDSEPEAEPGS

SEQ ID NO: 618 - protein, 20 aa, synthetic construct
  SOURCE 1..20
PPPPPEESSDSEPEAEPGSP

SEQ ID NO: 619 - protein, 20 aa, synthetic construct
  SOURCE 1..20
PPPPEESSDSEPEAEPGSPQ

SEQ ID NO: 620 - protein, 20 aa, synthetic construct
  SOURCE 1..20
PPPEESSDSEPEAEPGSPQK

SEQ ID NO: 621 - protein, 21 aa, synthetic construct
  SOURCE 1..21
SDPEPPDAGEDSKSENGENAP

SEQ ID NO: 622 - protein, 20 aa, synthetic construct
  SOURCE 1..20
SDSESEDPPRNQASDSENEE

SEQ ID NO: 623 - protein, 21 aa, synthetic construct
  SOURCE 1..21
GPGEDAEPDEDPQSEDSEAPS

SEQ ID NO: 624 - protein, 21 aa, synthetic construct
  SOURCE 1..21
PGEDAEPDEDPQSEDSEAPSS

SEQ ID NO: 625 - protein, 22 aa, synthetic construct
  SOURCE 1..22
GPGEDAEPDEDPQSEDSEAPSS

SEQ ID NO: 626 - protein, 23 aa, synthetic construct
  SOURCE 1..23
ESESSSSDSEANEPSQSASPEPE

SEQ ID NO: 627 - protein, 25 aa, synthetic construct
  SOURCE 1..25
DSESESSSSDSEANEPSQSASPEPE

SEQ ID NO: 628 - protein, 26 aa, synthetic construct
  SOURCE 1..26
SDSESESSSSDSEANEPSQSASPEPE

SEQ ID NO: 629 - protein, 26 aa, synthetic construct
  SOURCE 1..26
DSESESSSSDSEANEPSQSASPEPEP

SEQ ID NO: 630 - protein, 23 aa, synthetic construct
  SOURCE 1..23
HQEDSEEESQEEEAEGASEPPPP

SEQ ID NO: 631 - protein, 25 aa, synthetic construct
  SOURCE 1..25
GDHQEDSEEESQEEEAEGASEPPPP

SEQ ID NO: 632 - protein, 20 aa, synthetic construct
  SOURCE 1..20
PSQPPEEPEPDEAESSPDPQ

SEQ ID NO: 633 - protein, 21 aa, synthetic construct
  SOURCE 1..21
DPAPSQPPEEPEPDEAESSPD

SEQ ID NO: 634 - protein, 21 aa, synthetic construct
  SOURCE 1..21
PAPSQPPEEPEPDEAESSPDP

SEQ ID NO: 635 - protein, 21 aa, synthetic construct
  SOURCE 1..21
APSQPPEEPEPDEAESSPDPQ

SEQ ID NO: 636 - protein, 21 aa, synthetic construct
  SOURCE 1..21
PSQPPEEPEPDEAESSPDPQA

SEQ ID NO: 637 - protein, 22 aa, synthetic construct
  SOURCE 1..22
DPAPSQPPEEPEPDEAESSPDP

SEQ ID NO: 638 - protein, 22 aa, synthetic construct
  SOURCE 1..22
PAPSQPPEEPEPDEAESSPDPQ

SEQ ID NO: 639 - protein, 23 aa, synthetic construct
  SOURCE 1..23
DPAPSQPPEEPEPDEAESSPDPQ

SEQ ID NO: 640 - protein, 21 aa, synthetic construct
  SOURCE 1..21
PGSQPQASSGPEAEEEEEDDE

SEQ ID NO: 641 - protein, 20 aa, synthetic construct
  SOURCE 1..20
DSPDSQEEQKGESSASSPEE

SEQ ID NO: 642 - protein, 20 aa, synthetic construct
  SOURCE 1..20
SPDSQEEQKGESSASSPEEP

SEQ ID NO: 643 - protein, 20 aa, synthetic construct
  SOURCE 1..20
PDSQEEQKGESSASSPEEPE

SEQ ID NO: 644 - protein, 20 aa, synthetic construct
  SOURCE 1..20
DSQEEQKGESSASSPEEPEE

SEQ ID NO: 645 - protein, 21 aa, synthetic construct
  SOURCE 1..21
DSPDSQEEQKGESSASSPEEP

SEQ ID NO: 646 - protein, 21 aa, synthetic construct
  SOURCE 1..21
SPDSQEEQKGESSASSPEEPE

SEQ ID NO: 647 - protein, 21 aa, synthetic construct
  SOURCE 1..21
PDSQEEQKGESSASSPEEPEE

SEQ ID NO: 648 - protein, 22 aa, synthetic construct
  SOURCE 1..22
PADSPDSQEEQKGESSASSPEE

SEQ ID NO: 649 - protein, 22 aa, synthetic construct
  SOURCE 1..22
ADSPDSQEEQKGESSASSPEEP

SEQ ID NO: 650 - protein, 22 aa, synthetic construct
  SOURCE 1..22
DSPDSQEEQKGESSASSPEEPE

SEQ ID NO: 651 - protein, 22 aa, synthetic construct
  SOURCE 1..22
SPDSQEEQKGESSASSPEEPEE

SEQ ID NO: 652 - protein, 23 aa, synthetic construct
  SOURCE 1..23
PADSPDSQEEQKGESSASSPEEP

SEQ ID NO: 653 - protein, 23 aa, synthetic construct
  SOURCE 1..23
ADSPDSQEEQKGESSASSPEEPE

SEQ ID NO: 654 - protein, 23 aa, synthetic construct
  SOURCE 1..23
DSPDSQEEQKGESSASSPEEPEE

SEQ ID NO: 655 - protein, 24 aa, synthetic construct
  SOURCE 1..24
PADSPDSQEEQKGESSASSPEEPE

SEQ ID NO: 656 - protein, 24 aa, synthetic construct
  SOURCE 1..24
ADSPDSQEEQKGESSASSPEEPEE

SEQ ID NO: 657 - protein, 25 aa, synthetic construct
  SOURCE 1..25
PADSPDSQEEQKGESSASSPEEPEE

SEQ ID NO: 658 - protein, 20 aa, synthetic construct
  SOURCE 1..20
SPSPEDESSSSSSSSSSEDE

SEQ ID NO: 659 - protein, 20 aa, synthetic construct
  SOURCE 1..20
PSPEDESSSSSSSSSSEDEE

SEQ ID NO: 660 - protein, 23 aa, synthetic construct
  SOURCE 1..23
PRSPSPEDESSSSSSSSSSEDEE

SEQ ID NO: 661 - protein, 24 aa, synthetic construct
  SOURCE 1..24
PRSPSPEDESSSSSSSSSSEDEEE

SEQ ID NO: 662 - protein, 20 aa, synthetic construct
  SOURCE 1..20
SSSDSSDSDSSEDDEAPSKP

SEQ ID NO: 663 - protein, 21 aa, synthetic construct
  SOURCE 1..21
PSPGSPRGQPQDQDDDEDDEE

SEQ ID NO: 664 - protein, 20 aa, synthetic construct
  SOURCE 1..20
QQAEDHPQNPPEDPNQDPPE

SEQ ID NO: 665 - protein, 20 aa, synthetic construct
  SOURCE 1..20
QAEDHPQNPPEDPNQDPPED

SEQ ID NO: 666 - protein, 20 aa, synthetic construct
  SOURCE 1..20
AEDHPQNPPEDPNQDPPEDD

SEQ ID NO: 667 - protein, 20 aa, synthetic construct
  SOURCE 1..20
EDHPQNPPEDPNQDPPEDDS

SEQ ID NO: 668 - protein, 21 aa, synthetic construct
  SOURCE 1..21
QQAEDHPQNPPEDPNQDPPED

SEQ ID NO: 669 - protein, 21 aa, synthetic construct
  SOURCE 1..21
QAEDHPQNPPEDPNQDPPEDD

SEQ ID NO: 670 - protein, 21 aa, synthetic construct
  SOURCE 1..21
AEDHPQNPPEDPNQDPPEDDS

SEQ ID NO: 671 - protein, 22 aa, synthetic construct
  SOURCE 1..22
PQQAEDHPQNPPEDPNQDPPED

SEQ ID NO: 672 - protein, 22 aa, synthetic construct
  SOURCE 1..22
QQAEDHPQNPPEDPNQDPPEDD

SEQ ID NO: 673 - protein, 22 aa, synthetic construct
  SOURCE 1..22
QAEDHPQNPPEDPNQDPPEDDS

SEQ ID NO: 674 - protein, 23 aa, synthetic construct
  SOURCE 1..23
DGEAGPQQAEDHPQNPPEDPNQD

SEQ ID NO: 675 - protein, 23 aa, synthetic construct
  SOURCE 1..23
GPQQAEDHPQNPPEDPNQDPPED

SEQ ID NO: 676 - protein, 23 aa, synthetic construct
  SOURCE 1..23
PQQAEDHPQNPPEDPNQDPPEDD

SEQ ID NO: 677 - protein, 23 aa, synthetic construct
  SOURCE 1..23
QQAEDHPQNPPEDPNQDPPEDDS

SEQ ID NO: 678 - protein, 24 aa, synthetic construct
  SOURCE 1..24
GPQQAEDHPQNPPEDPNQDPPEDD

SEQ ID NO: 679 - protein, 24 aa, synthetic construct
  SOURCE 1..24
PQQAEDHPQNPPEDPNQDPPEDDS

SEQ ID NO: 680 - protein, 25 aa, synthetic construct
  SOURCE 1..25
EAGPQQAEDHPQNPPEDPNQDPPED

SEQ ID NO: 681 - protein, 25 aa, synthetic construct
  SOURCE 1..25
AGPQQAEDHPQNPPEDPNQDPPEDD

SEQ ID NO: 682 - protein, 25 aa, synthetic construct
  SOURCE 1..25
GPQQAEDHPQNPPEDPNQDPPEDDS

SEQ ID NO: 683 - protein, 26 aa, synthetic construct
  SOURCE 1..26
DGEAGPQQAEDHPQNPPEDPNQDPPE

SEQ ID NO: 684 - protein, 26 aa, synthetic construct
  SOURCE 1..26
GEAGPQQAEDHPQNPPEDPNQDPPED

SEQ ID NO: 685 - protein, 26 aa, synthetic construct
  SOURCE 1..26
EAGPQQAEDHPQNPPEDPNQDPPEDD

SEQ ID NO: 686 - protein, 26 aa, synthetic construct
  SOURCE 1..26
AGPQQAEDHPQNPPEDPNQDPPEDDS

SEQ ID NO: 687 - protein, 27 aa, synthetic construct
  SOURCE 1..27
DGEAGPQQAEDHPQNPPEDPNQDPPED

SEQ ID NO: 688 - protein, 27 aa, synthetic construct
  SOURCE 1..27
GEAGPQQAEDHPQNPPEDPNQDPPEDD

SEQ ID NO: 689 - protein, 27 aa, synthetic construct
  SOURCE 1..27
EAGPQQAEDHPQNPPEDPNQDPPEDDS

SEQ ID NO: 690 - protein, 28 aa, synthetic construct
  SOURCE 1..28
DGEAGPQQAEDHPQNPPEDPNQDPPEDD

SEQ ID NO: 691 - protein, 28 aa, synthetic construct
  SOURCE 1..28
GEAGPQQAEDHPQNPPEDPNQDPPEDDS

SEQ ID NO: 692 - protein, 29 aa, synthetic construct
  SOURCE 1..29
DGEAGPQQAEDHPQNPPEDPNQDPPEDDS

SEQ ID NO: 693 - protein, 31 aa, synthetic construct
  SOURCE 1..31
PAGDGEAGPQQAEDHPQNPPEDPNQDPPEDD

SEQ ID NO: 694 - protein, 31 aa, synthetic construct
  SOURCE 1..31
AGDGEAGPQQAEDHPQNPPEDPNQDPPEDDS

SEQ ID NO: 695 - protein, 32 aa, synthetic construct
  SOURCE 1..32
PAGDGEAGPQQAEDHPQNPPEDPNQDPPEDDS

SEQ ID NO: 696 - protein, 20 aa, synthetic construct
  SOURCE 1..20
QNQKEAEEPGPDSENSQENP

SEQ ID NO: 697 - protein, 20 aa, synthetic construct
  SOURCE 1..20
NQKEAEEPGPDSENSQENPP

SEQ ID NO: 698 - protein, 20 aa, synthetic construct
  SOURCE 1..20
DQNESQSPQEPEEGPSEDDK

SEQ ID NO: 699 - protein, 20 aa, synthetic construct
  SOURCE 1..20
QNESQSPQEPEEGPSEDDKA

SEQ ID NO: 700 - protein, 20 aa, synthetic construct
  SOURCE 1..20
NESQSPQEPEEGPSEDDKAE

SEQ ID NO: 701 - protein, 21 aa, synthetic construct
  SOURCE 1..21
DQNESQSPQEPEEGPSEDDKA

SEQ ID NO: 702 - protein, 21 aa, synthetic construct
  SOURCE 1..21
QNESQSPQEPEEGPSEDDKAE

SEQ ID NO: 703 - protein, 21 aa, synthetic construct
  SOURCE 1..21
NESQSPQEPEEGPSEDDKAEG

SEQ ID NO: 704 - protein, 21 aa, synthetic construct
  SOURCE 1..21
ESQSPQEPEEGPSEDDKAEGE

SEQ ID NO: 705 - protein, 21 aa, synthetic construct
  SOURCE 1..21
SQSPQEPEEGPSEDDKAEGEE

SEQ ID NO: 706 - protein, 22 aa, synthetic construct
  SOURCE 1..22
DQNESQSPQEPEEGPSEDDKAE

SEQ ID NO: 707 - protein, 22 aa, synthetic construct
  SOURCE 1..22
QNESQSPQEPEEGPSEDDKAEG

SEQ ID NO: 708 - protein, 22 aa, synthetic construct
  SOURCE 1..22
NESQSPQEPEEGPSEDDKAEGE

SEQ ID NO: 709 - protein, 23 aa, synthetic construct
  SOURCE 1..23
DQNESQSPQEPEEGPSEDDKAEG

SEQ ID NO: 710 - protein, 23 aa, synthetic construct
  SOURCE 1..23
QNESQSPQEPEEGPSEDDKAEGE

SEQ ID NO: 711 - protein, 23 aa, synthetic construct
  SOURCE 1..23
NESQSPQEPEEGPSEDDKAEGEE

SEQ ID NO: 712 - protein, 24 aa, synthetic construct
  SOURCE 1..24
DQNESQSPQEPEEGPSEDDKAEGE

SEQ ID NO: 713 - protein, 24 aa, synthetic construct
  SOURCE 1..24
QNESQSPQEPEEGPSEDDKAEGEE

SEQ ID NO: 714 - protein, 25 aa, synthetic construct
  SOURCE 1..25
DQNESQSPQEPEEGPSEDDKAEGEE

SEQ ID NO: 715 - protein, 25 aa, synthetic construct
  SOURCE 1..25
QNESQSPQEPEEGPSEDDKAEGEEE

SEQ ID NO: 716 - protein, 21 aa, synthetic construct
  SOURCE 1..21
XEASSSEEEPPSPDDKENQAP

SEQ ID NO: 717 - protein, 21 aa, synthetic construct
  SOURCE 1..21
PASSSSNPEEGPEEDREAESE

SEQ ID NO: 718 - protein, 20 aa, synthetic construct
  SOURCE 1..20
DKPEEEDDEAQQPQPQSGPE

SEQ ID NO: 719 - protein, 20 aa, synthetic construct
  SOURCE 1..20
KPEEEDDEAQQPQPQSGPEE

SEQ ID NO: 720 - protein, 21 aa, synthetic construct
  SOURCE 1..21
AGEGDKPEEEDDEAQQPQPQS

SEQ ID NO: 721 - protein, 21 aa, synthetic construct
  SOURCE 1..21
EGDKPEEEDDEAQQPQPQSGP

SEQ ID NO: 722 - protein, 21 aa, synthetic construct
  SOURCE 1..21
GDKPEEEDDEAQQPQPQSGPE

SEQ ID NO: 723 - protein, 21 aa, synthetic construct
  SOURCE 1..21
DKPEEEDDEAQQPQPQSGPEE

SEQ ID NO: 724 - protein, 21 aa, synthetic construct
  SOURCE 1..21
KPEEEDDEAQQPQPQSGPEEA

SEQ ID NO: 725 - protein, 21 aa, synthetic construct
  SOURCE 1..21
PEEEDDEAQQPQPQSGPEEAE

SEQ ID NO: 726 - protein, 21 aa, synthetic construct
  SOURCE 1..21
EEDDEAQQPQPQSGPEEAEEG

SEQ ID NO: 727 - protein, 21 aa, synthetic construct
  SOURCE 1..21
EDDEAQQPQPQSGPEEAEEGE

SEQ ID NO: 728 - protein, 21 aa, synthetic construct
  SOURCE 1..21
DDEAQQPQPQSGPEEAEEGEE

SEQ ID NO: 729 - protein, 21 aa, synthetic construct
  SOURCE 1..21
DEAQQPQPQSGPEEAEEGEEE

SEQ ID NO: 730 - protein, 21 aa, synthetic construct
  SOURCE 1..21
EAQQPQPQSGPEEAEEGEEEE

SEQ ID NO: 731 - protein, 21 aa, synthetic construct
  SOURCE 1..21
QQPQPQSGPEEAEEGEEEEAE

SEQ ID NO: 732 - protein, 21 aa, synthetic construct
  SOURCE 1..21
QPQPQSGPEEAEEGEEEEAER

SEQ ID NO: 733 - protein, 22 aa, synthetic construct
  SOURCE 1..22
EGDKPEEEDDEAQQPQPQSGPE

SEQ ID NO: 734 - protein, 22 aa, synthetic construct
  SOURCE 1..22
GDKPEEEDDEAQQPQPQSGPEE

SEQ ID NO: 735 - protein, 22 aa, synthetic construct
  SOURCE 1..22
DKPEEEDDEAQQPQPQSGPEEA

SEQ ID NO: 736 - protein, 22 aa, synthetic construct
  SOURCE 1..22
KPEEEDDEAQQPQPQSGPEEAE

SEQ ID NO: 737 - protein, 22 aa, synthetic construct
  SOURCE 1..22
QQPQPQSGPEEAEEGEEEEAER

SEQ ID NO: 738 - protein, 23 aa, synthetic construct
  SOURCE 1..23
EGDKPEEEDDEAQQPQPQSGPEE

SEQ ID NO: 739 - protein, 23 aa, synthetic construct
  SOURCE 1..23
GDKPEEEDDEAQQPQPQSGPEEA

SEQ ID NO: 740 - protein, 23 aa, synthetic construct
  SOURCE 1..23
DKPEEEDDEAQQPQPQSGPEEAE

SEQ ID NO: 741 - protein, 23 aa, synthetic construct
  SOURCE 1..23
KPEEEDDEAQQPQPQSGPEEAEE

SEQ ID NO: 742 - protein, 23 aa, synthetic construct
  SOURCE 1..23
PEEEDDEAQQPQPQSGPEEAEEG

SEQ ID NO: 743 - protein, 24 aa, synthetic construct
  SOURCE 1..24
EGDKPEEEDDEAQQPQPQSGPEEA

SEQ ID NO: 744 - protein, 24 aa, synthetic construct
  SOURCE 1..24
GDKPEEEDDEAQQPQPQSGPEEAE

SEQ ID NO: 745 - protein, 24 aa, synthetic construct
  SOURCE 1..24
KPEEEDDEAQQPQPQSGPEEAEEG

SEQ ID NO: 746 - protein, 25 aa, synthetic construct
  SOURCE 1..25
EGDKPEEEDDEAQQPQPQSGPEEAE

SEQ ID NO: 747 - protein, 25 aa, synthetic construct
  SOURCE 1..25
GDKPEEEDDEAQQPQPQSGPEEAEE

SEQ ID NO: 748 - protein, 25 aa, synthetic construct
  SOURCE 1..25
DKPEEEDDEAQQPQPQSGPEEAEEG

SEQ ID NO: 749 - protein, 25 aa, synthetic construct
  SOURCE 1..25
KPEEEDDEAQQPQPQSGPEEAEEGE

SEQ ID NO: 750 - protein, 20 aa, synthetic construct
  SOURCE 1..20
PEEEHAPGEDESSPQPSQPS

SEQ ID NO: 751 - protein, 20 aa, synthetic construct
  SOURCE 1..20
XPPPEESSDSEPEAEPGSPQ

SEQ ID NO: 752 - protein, 20 aa, synthetic construct
  SOURCE 1..20
PPPEESSDSEPEAEPGSPQK

SEQ ID NO: 753 - protein, 20 aa, synthetic construct
  SOURCE 1..20
KEPKEEKKDDDEEAPKPSSD

SEQ ID NO: 754 - protein, 20 aa, synthetic construct
  SOURCE 1..20
SEEEKPPEEDKEEEEEKKAP

SEQ ID NO: 755 - protein, 21 aa, synthetic construct
  SOURCE 1..21
PAEEDEDDPEQEKEAGEPGRP

SEQ ID NO: 756 - protein, 20 aa, synthetic construct
  SOURCE 1..20
PEPEPEPEPEPEPAPEPEPE

SEQ ID NO: 757 - protein, 20 aa, synthetic construct
  SOURCE 1..20
EPEPEPEPEPEPAPEPEPEP

SEQ ID NO: 758 - protein, 20 aa, synthetic construct
  SOURCE 1..20
DEDPEEDGSPDPEPSPEPEP

SEQ ID NO: 759 - protein, 20 aa, synthetic construct
  SOURCE 1..20
EDPEEDGSPDPEPSPEPEPK

SEQ ID NO: 760 - protein, 21 aa, synthetic construct
  SOURCE 1..21
DEDPEEDGSPDPEPSPEPEPK

SEQ ID NO: 761 - protein, 22 aa, synthetic construct
  SOURCE 1..22
DEDPEEDGSPDPEPSPEPEPKP

SEQ ID NO: 762 - protein, 20 aa, synthetic construct
  SOURCE 1..20
KPEDKDPRDPEESKEPKEEK

SEQ ID NO: 763 - protein, 20 aa, synthetic construct
  SOURCE 1..20
PEDKDPRDPEESKEPKEEKQ

SEQ ID NO: 764 - protein, 20 aa, synthetic construct
  SOURCE 1..20
EDKDPRDPEESKEPKEEKQR

SEQ ID NO: 765 - protein, 20 aa, synthetic construct
  SOURCE 1..20
KRNDSEEEERERDEEQEPPP

SEQ ID NO: 766 - protein, 20 aa, synthetic construct
  SOURCE 1..20
PEEEPDDQDAPDEHEPSPSE

SEQ ID NO: 767 - protein, 20 aa, synthetic construct
  SOURCE 1..20
EEEPDDQDAPDEHEPSPSED

SEQ ID NO: 768 - protein, 21 aa, synthetic construct
  SOURCE 1..21
PEEEPDDQDAPDEHEPSPSED

SEQ ID NO: 769 - protein, 21 aa, synthetic construct
  SOURCE 1..21
EEEPDDQDAPDEHEPSPSEDA

SEQ ID NO: 770 - protein, 21 aa, synthetic construct
  SOURCE 1..21
EEPDDQDAPDEHEPSPSEDAP

SEQ ID NO: 771 - protein, 22 aa, synthetic construct
  SOURCE 1..22
PEEEPDDQDAPDEHEPSPSEDA

SEQ ID NO: 772 - protein, 22 aa, synthetic construct
  SOURCE 1..22
EEEPDDQDAPDEHEPSPSEDAP

SEQ ID NO: 773 - protein, 23 aa, synthetic construct
  SOURCE 1..23
PEEEPDDQDAPDEHEPSPSEDAP

SEQ ID NO: 774 - protein, 20 aa, synthetic construct
  SOURCE 1..20
SPAPSPDSDSDSDSDGEEEE

SEQ ID NO: 775 - protein, 20 aa, synthetic construct
  SOURCE 1..20
PAPSPDSDSDSDSDGEEEEE

SEQ ID NO: 776 - protein, 22 aa, synthetic construct
  SOURCE 1..22
PSPAPSPDSDSDSDSDGEEEEE

SEQ ID NO: 777 - protein, 23 aa, synthetic construct
  SOURCE 1..23
PSPAPSPDSDSDSDSDGEEEEEE

SEQ ID NO: 778 - protein, 24 aa, synthetic construct
  SOURCE 1..24
APSPAPSPDSDSDSDSDGEEEEEE

SEQ ID NO: 779 - protein, 24 aa, synthetic construct
  SOURCE 1..24
PSPAPSPDSDSDSDSDGEEEEEEE

SEQ ID NO: 780 - protein, 25 aa, synthetic construct
  SOURCE 1..25
APSPAPSPDSDSDSDSDGEEEEEEE

SEQ ID NO: 781 - protein, 25 aa, synthetic construct
  SOURCE 1..25
PSPAPSPDSDSDSDSDGEEEEEEEG

SEQ ID NO: 782 - protein, 26 aa, synthetic construct
  SOURCE 1..26
GAPSPAPSPDSDSDSDSDGEEEEEEE

SEQ ID NO: 783 - protein, 26 aa, synthetic construct
  SOURCE 1..26
APSPAPSPDSDSDSDSDGEEEEEEEG

SEQ ID NO: 784 - protein, 26 aa, synthetic construct
  SOURCE 1..26
PSPAPSPDSDSDSDSDGEEEEEEEGE

SEQ ID NO: 785 - protein, 21 aa, synthetic construct
  SOURCE 1..21
EKNDEDEPQKPEDKGDPEGPE

SEQ ID NO: 786 - protein, 22 aa, synthetic construct
  SOURCE 1..22
EKNDEDEPQKPEDKGDPEGPEA

SEQ ID NO: 787 - protein, 20 aa, synthetic construct
  SOURCE 1..20
EDEEEEEEEEEEEDEGPAPP

SEQ ID NO: 788 - protein, 20 aa, synthetic construct
  SOURCE 1..20
DEEEEEEEEEEEDEGPAPPS

SEQ ID NO: 789 - protein, 20 aa, synthetic construct
  SOURCE 1..20
EREPDPPDDRDASDGEDEKP

SEQ ID NO: 790 - protein, 20 aa, synthetic construct
  SOURCE 1..20
REPDPPDDRDASDGEDEKPP

SEQ ID NO: 791 - protein, 21 aa, synthetic construct
  SOURCE 1..21
GEREPDPPDDRDASDGEDEKP

SEQ ID NO: 792 - protein, 21 aa, synthetic construct
  SOURCE 1..21
EREPDPPDDRDASDGEDEKPP

SEQ ID NO: 793 - protein, 22 aa, synthetic construct
  SOURCE 1..22
EGEREPDPPDDRDASDGEDEKP

SEQ ID NO: 794 - protein, 22 aa, synthetic construct
  SOURCE 1..22
GEREPDPPDDRDASDGEDEKPP

SEQ ID NO: 795 - protein, 23 aa, synthetic construct
  SOURCE 1..23
EGEREPDPPDDRDASDGEDEKPP

SEQ ID NO: 796 - protein, 22 aa, synthetic construct
  SOURCE 1..22
EEEEEQPGKAPDPQDPQDAESD

SEQ ID NO: 797 - protein, 20 aa, synthetic construct
  SOURCE 1..20
QEPEEKQEPEEKQEPEEKQK

SEQ ID NO: 798 - protein, 20 aa, synthetic construct
  SOURCE 1..20
EPEEKQEPEEKQEPEEKQKP

SEQ ID NO: 799 - protein, 20 aa, synthetic construct
  SOURCE 1..20
PEEKQEPEEKQEPEEKQKPE

SEQ ID NO: 800 - protein, 20 aa, synthetic construct
  SOURCE 1..20
EEKQEPEEKQEPEEKQKPEA

SEQ ID NO: 801 - protein, 21 aa, synthetic construct
  SOURCE 1..21
EPEEKQEPEEKQEPEEKQKPE

SEQ ID NO: 802 - protein, 22 aa, synthetic construct
  SOURCE 1..22
QEPEEKQEPEEKQEPEEKQKPE

SEQ ID NO: 803 - protein, 22 aa, synthetic construct
  SOURCE 1..22
EPEEKQEPEEKQEPEEKQKPEA

SEQ ID NO: 804 - protein, 20 aa, synthetic construct
  SOURCE 1..20
AGDDDDDDDDSPDPESPDDS

SEQ ID NO: 805 - protein, 20 aa, synthetic construct
  SOURCE 1..20
GDDDDDDDDSPDPESPDDSE

SEQ ID NO: 806 - protein, 20 aa, synthetic construct
  SOURCE 1..20
DDDDDDDDSPDPESPDDSES

SEQ ID NO: 807 - protein, 20 aa, synthetic construct
  SOURCE 1..20
DDDDDDDSPDPESPDDSESD

SEQ ID NO: 808 - protein, 20 aa, synthetic construct
  SOURCE 1..20
DDDDDDSPDPESPDDSESDS

SEQ ID NO: 809 - protein, 20 aa, synthetic construct
  SOURCE 1..20
DDDDDSPDPESPDDSESDSE

SEQ ID NO: 810 - protein, 20 aa, synthetic construct
  SOURCE 1..20
DDDDSPDPESPDDSESDSES

SEQ ID NO: 811 - protein, 20 aa, synthetic construct
  SOURCE 1..20
DDDSPDPESPDDSESDSESE

SEQ ID NO: 812 - protein, 20 aa, synthetic construct
  SOURCE 1..20
DDSPDPESPDDSESDSESEK

SEQ ID NO: 813 - protein, 20 aa, synthetic construct
  SOURCE 1..20
DSPDPESPDDSESDSESEKE

SEQ ID NO: 814 - protein, 20 aa, synthetic construct
  SOURCE 1..20
SPDPESPDDSESDSESEKEE

SEQ ID NO: 815 - protein, 20 aa, synthetic construct
  SOURCE 1..20
PDPESPDDSESDSESEKEES

SEQ ID NO: 816 - protein, 21 aa, synthetic construct
  SOURCE 1..21
DPDQPREDPAEEEKEEKDAPE

SEQ ID NO: 817 - protein, 20 aa, synthetic construct
  SOURCE 1..20
EGKPENESEPKHEEEPKPEE

SEQ ID NO: 818 - protein, 20 aa, synthetic construct
  SOURCE 1..20
PENESEPKHEEEPKPEEKPE

SEQ ID NO: 819 - protein, 20 aa, synthetic construct
  SOURCE 1..20
ENESEPKHEEEPKPEEKPEE

SEQ ID NO: 820 - protein, 20 aa, synthetic construct
  SOURCE 1..20
NESEPKHEEEPKPEEKPEEE

SEQ ID NO: 821 - protein, 20 aa, synthetic construct
  SOURCE 1..20
ESEPKHEEEPKPEEKPEEEE

SEQ ID NO: 822 - protein, 20 aa, synthetic construct
  SOURCE 1..20
SEPKHEEEPKPEEKPEEEEK

SEQ ID NO: 823 - protein, 21 aa, synthetic construct
  SOURCE 1..21
PENESEPKHEEEPKPEEKPEE

SEQ ID NO: 824 - protein, 21 aa, synthetic construct
  SOURCE 1..21
ENESEPKHEEEPKPEEKPEEE

SEQ ID NO: 825 - protein, 21 aa, synthetic construct
  SOURCE 1..21
NESEPKHEEEPKPEEKPEEEE

SEQ ID NO: 826 - protein, 21 aa, synthetic construct
  SOURCE 1..21
ESEPKHEEEPKPEEKPEEEEK

SEQ ID NO: 827 - protein, 22 aa, synthetic construct
  SOURCE 1..22
KPENESEPKHEEEPKPEEKPEE

SEQ ID NO: 828 - protein, 22 aa, synthetic construct
  SOURCE 1..22
PENESEPKHEEEPKPEEKPEEE

SEQ ID NO: 829 - protein, 22 aa, synthetic construct
  SOURCE 1..22
ENESEPKHEEEPKPEEKPEEEE

SEQ ID NO: 830 - protein, 22 aa, synthetic construct
  SOURCE 1..22
NESEPKHEEEPKPEEKPEEEEK

SEQ ID NO: 831 - protein, 23 aa, synthetic construct
  SOURCE 1..23
KPENESEPKHEEEPKPEEKPEEE

SEQ ID NO: 832 - protein, 23 aa, synthetic construct
  SOURCE 1..23
PENESEPKHEEEPKPEEKPEEEE

SEQ ID NO: 833 - protein, 23 aa, synthetic construct
  SOURCE 1..23
ENESEPKHEEEPKPEEKPEEEEK

SEQ ID NO: 834 - protein, 24 aa, synthetic construct
  SOURCE 1..24
EGKPENESEPKHEEEPKPEEKPEE

SEQ ID NO: 835 - protein, 24 aa, synthetic construct
  SOURCE 1..24
GKPENESEPKHEEEPKPEEKPEEE

SEQ ID NO: 836 - protein, 24 aa, synthetic construct
  SOURCE 1..24
KPENESEPKHEEEPKPEEKPEEEE

SEQ ID NO: 837 - protein, 24 aa, synthetic construct
  SOURCE 1..24
PENESEPKHEEEPKPEEKPEEEEK

SEQ ID NO: 838 - protein, 25 aa, synthetic construct
  SOURCE 1..25
EGKPENESEPKHEEEPKPEEKPEEE

SEQ ID NO: 839 - protein, 25 aa, synthetic construct
  SOURCE 1..25
GKPENESEPKHEEEPKPEEKPEEEE

SEQ ID NO: 840 - protein, 25 aa, synthetic construct
  SOURCE 1..25
KPENESEPKHEEEPKPEEKPEEEEK

SEQ ID NO: 841 - protein, 26 aa, synthetic construct
  SOURCE 1..26
EGKPENESEPKHEEEPKPEEKPEEEE

SEQ ID NO: 842 - protein, 26 aa, synthetic construct
  SOURCE 1..26
GKPENESEPKHEEEPKPEEKPEEEEK

SEQ ID NO: 843 - protein, 27 aa, synthetic construct
  SOURCE 1..27
EGKPENESEPKHEEEPKPEEKPEEEEK

SEQ ID NO: 844 - protein, 20 aa, synthetic construct
  SOURCE 1..20
KPPEEDPEEQAEENPEGEQP

SEQ ID NO: 845 - protein, 20 aa, synthetic construct
  SOURCE 1..20
PPEEDPEEQAEENPEGEQPE

SEQ ID NO: 846 - protein, 20 aa, synthetic construct
  SOURCE 1..20
PEEDPEEQAEENPEGEQPEE

SEQ ID NO: 847 - protein, 21 aa, synthetic construct
  SOURCE 1..21
KPPEEDPEEQAEENPEGEQPE

SEQ ID NO: 848 - protein, 21 aa, synthetic construct
  SOURCE 1..21
PPEEDPEEQAEENPEGEQPEE

SEQ ID NO: 849 - protein, 22 aa, synthetic construct
  SOURCE 1..22
KPPEEDPEEQAEENPEGEQPEE

SEQ ID NO: 850 - protein, 20 aa, synthetic construct
  SOURCE 1..20
PDDDDESEDHDDPDNAHESP

SEQ ID NO: 851 - protein, 20 aa, synthetic construct
  SOURCE 1..20
GEPEPEPEPEPEPEPESEPE

SEQ ID NO: 852 - protein, 20 aa, synthetic construct
  SOURCE 1..20
EPEPEPEPEPEPEPESEPEP

SEQ ID NO: 853 - protein, 20 aa, synthetic construct
  SOURCE 1..20
PEPEPEPEPEPEPESEPEPE

SEQ ID NO: 854 - protein, 20 aa, synthetic construct
  SOURCE 1..20
EPEPEPEPEPEPESEPEPEP

SEQ ID NO: 855 - protein, 20 aa, synthetic construct
  SOURCE 1..20
PEPEPEPEPEPESEPEPEPE

SEQ ID NO: 856 - protein, 21 aa, synthetic construct
  SOURCE 1..21
GGEPEPEPEPEPEPEPESEPE

SEQ ID NO: 857 - protein, 21 aa, synthetic construct
  SOURCE 1..21
GEPEPEPEPEPEPEPESEPEP

SEQ ID NO: 858 - protein, 21 aa, synthetic construct
  SOURCE 1..21
EPEPEPEPEPEPEPESEPEPE

SEQ ID NO: 859 - protein, 21 aa, synthetic construct
  SOURCE 1..21
PEPEPEPEPEPEPESEPEPEP

SEQ ID NO: 860 - protein, 21 aa, synthetic construct
  SOURCE 1..21
EPEPEPEPEPEPESEPEPEPE

SEQ ID NO: 861 - protein, 22 aa, synthetic construct
  SOURCE 1..22
GGEPEPEPEPEPEPEPESEPEP

SEQ ID NO: 862 - protein, 22 aa, synthetic construct
  SOURCE 1..22
GEPEPEPEPEPEPEPESEPEPE

SEQ ID NO: 863 - protein, 22 aa, synthetic construct
  SOURCE 1..22
EPEPEPEPEPEPEPESEPEPEP

SEQ ID NO: 864 - protein, 22 aa, synthetic construct
  SOURCE 1..22
PEPEPEPEPEPEPESEPEPEPE

SEQ ID NO: 865 - protein, 23 aa, synthetic construct
  SOURCE 1..23
GGEPEPEPEPEPEPEPESEPEPE

SEQ ID NO: 866 - protein, 23 aa, synthetic construct
  SOURCE 1..23
GEPEPEPEPEPEPEPESEPEPEP

SEQ ID NO: 867 - protein, 23 aa, synthetic construct
  SOURCE 1..23
EPEPEPEPEPEPEPESEPEPEPE

SEQ ID NO: 868 - protein, 24 aa, synthetic construct
  SOURCE 1..24
GGEPEPEPEPEPEPEPESEPEPEP

SEQ ID NO: 869 - protein, 24 aa, synthetic construct
  SOURCE 1..24
GEPEPEPEPEPEPEPESEPEPEPE

SEQ ID NO: 870 - protein, 25 aa, synthetic construct
  SOURCE 1..25
GGEPEPEPEPEPEPEPESEPEPEPE

SEQ ID NO: 871 - protein, 20 aa, synthetic construct
  SOURCE 1..20
PEEEPDDQDAPDEHESPPPE

SEQ ID NO: 872 - protein, 20 aa, synthetic construct
  SOURCE 1..20
EEEPDDQDAPDEHESPPPED

SEQ ID NO: 873 - protein, 21 aa, synthetic construct
  SOURCE 1..21
PEEEPDDQDAPDEHESPPPED

SEQ ID NO: 874 - protein, 21 aa, synthetic construct
  SOURCE 1..21
EEEPDDQDAPDEHESPPPEDA

SEQ ID NO: 875 - protein, 21 aa, synthetic construct
  SOURCE 1..21
EEPDDQDAPDEHESPPPEDAP

SEQ ID NO: 876 - protein, 22 aa, synthetic construct
  SOURCE 1..22
PEEEPDDQDAPDEHESPPPEDA

SEQ ID NO: 877 - protein, 22 aa, synthetic construct
  SOURCE 1..22
EEEPDDQDAPDEHESPPPEDAP

SEQ ID NO: 878 - protein, 23 aa, synthetic construct
  SOURCE 1..23
PEEEPDDQDAPDEHESPPPEDAP

SEQ ID NO: 879 - protein, 20 aa, synthetic construct
  SOURCE 1..20
GPSSDDENEEESKPEKEDEP

SEQ ID NO: 880 - protein, 20 aa, synthetic construct
  SOURCE 1..20
PSSDDENEEESKPEKEDEPQ

SEQ ID NO: 881 - protein, 20 aa, synthetic construct
  SOURCE 1..20
SDDSDSEKRRPEEQEEEPQP

SEQ ID NO: 882 - protein, 20 aa, synthetic construct
  SOURCE 1..20
DDSDSEKRRPEEQEEEPQPR

SEQ ID NO: 883 - protein, 20 aa, synthetic construct
  SOURCE 1..20
DPREGEEEEEEDEPDPEAPE

SEQ ID NO: 884 - protein, 20 aa, synthetic construct
  SOURCE 1..20
PREGEEEEEEDEPDPEAPEN

SEQ ID NO: 885 - protein, 21 aa, synthetic construct
  SOURCE 1..21
DEEPGDPREGEEEEEEDEPDP

SEQ ID NO: 886 - protein, 21 aa, synthetic construct
  SOURCE 1..21
EEPGDPREGEEEEEEDEPDPE

SEQ ID NO: 887 - protein, 21 aa, synthetic construct
  SOURCE 1..21
EPGDPREGEEEEEEDEPDPEA

SEQ ID NO: 888 - protein, 21 aa, synthetic construct
  SOURCE 1..21
PGDPREGEEEEEEDEPDPEAP

SEQ ID NO: 889 - protein, 21 aa, synthetic construct
  SOURCE 1..21
GDPREGEEEEEEDEPDPEAPE

SEQ ID NO: 890 - protein, 21 aa, synthetic construct
  SOURCE 1..21
DPREGEEEEEEDEPDPEAPEN

SEQ ID NO: 891 - protein, 21 aa, synthetic construct
  SOURCE 1..21
PREGEEEEEEDEPDPEAPENG

SEQ ID NO: 892 - protein, 22 aa, synthetic construct
  SOURCE 1..22
EDEEPGDPREGEEEEEEDEPDP

SEQ ID NO: 893 - protein, 22 aa, synthetic construct
  SOURCE 1..22
DEEPGDPREGEEEEEEDEPDPE

SEQ ID NO: 894 - protein, 22 aa, synthetic construct
  SOURCE 1..22
EEPGDPREGEEEEEEDEPDPEA

SEQ ID NO: 895 - protein, 22 aa, synthetic construct
  SOURCE 1..22
EPGDPREGEEEEEEDEPDPEAP

SEQ ID NO: 896 - protein, 22 aa, synthetic construct
  SOURCE 1..22
PGDPREGEEEEEEDEPDPEAPE

SEQ ID NO: 897 - protein, 22 aa, synthetic construct
  SOURCE 1..22
GDPREGEEEEEEDEPDPEAPEN

SEQ ID NO: 898 - protein, 22 aa, synthetic construct
  SOURCE 1..22
DPREGEEEEEEDEPDPEAPENG

SEQ ID NO: 899 - protein, 22 aa, synthetic construct
  SOURCE 1..22
PREGEEEEEEDEPDPEAPENGS

SEQ ID NO: 900 - protein, 23 aa, synthetic construct
  SOURCE 1..23
PEEEDEEPGDPREGEEEEEEDEP

SEQ ID NO: 901 - protein, 23 aa, synthetic construct
  SOURCE 1..23
EEDEEPGDPREGEEEEEEDEPDP

SEQ ID NO: 902 - protein, 23 aa, synthetic construct
  SOURCE 1..23
EDEEPGDPREGEEEEEEDEPDPE

SEQ ID NO: 903 - protein, 23 aa, synthetic construct
  SOURCE 1..23
DEEPGDPREGEEEEEEDEPDPEA

SEQ ID NO: 904 - protein, 23 aa, synthetic construct
  SOURCE 1..23
EEPGDPREGEEEEEEDEPDPEAP

SEQ ID NO: 905 - protein, 23 aa, synthetic construct
  SOURCE 1..23
EPGDPREGEEEEEEDEPDPEAPE

SEQ ID NO: 906 - protein, 23 aa, synthetic construct
  SOURCE 1..23
PGDPREGEEEEEEDEPDPEAPEN

SEQ ID NO: 907 - protein, 23 aa, synthetic construct
  SOURCE 1..23
DPREGEEEEEEDEPDPEAPENGS

SEQ ID NO: 908 - protein, 24 aa, synthetic construct
  SOURCE 1..24
APEEEDEEPGDPREGEEEEEEDEP

SEQ ID NO: 909 - protein, 24 aa, synthetic construct
  SOURCE 1..24
PEEEDEEPGDPREGEEEEEEDEPD

SEQ ID NO: 910 - protein, 24 aa, synthetic construct
  SOURCE 1..24
EEEDEEPGDPREGEEEEEEDEPDP

SEQ ID NO: 911 - protein, 24 aa, synthetic construct
  SOURCE 1..24
EEDEEPGDPREGEEEEEEDEPDPE

SEQ ID NO: 912 - protein, 24 aa, synthetic construct
  SOURCE 1..24
EDEEPGDPREGEEEEEEDEPDPEA

SEQ ID NO: 913 - protein, 24 aa, synthetic construct
  SOURCE 1..24
DEEPGDPREGEEEEEEDEPDPEAP

SEQ ID NO: 914 - protein, 24 aa, synthetic construct
  SOURCE 1..24
EEPGDPREGEEEEEEDEPDPEAPE

SEQ ID NO: 915 - protein, 24 aa, synthetic construct
  SOURCE 1..24
EPGDPREGEEEEEEDEPDPEAPEN

SEQ ID NO: 916 - protein, 25 aa, synthetic construct
  SOURCE 1..25
AAPEEEDEEPGDPREGEEEEEEDEP

SEQ ID NO: 917 - protein, 25 aa, synthetic construct
  SOURCE 1..25
APEEEDEEPGDPREGEEEEEEDEPD

SEQ ID NO: 918 - protein, 25 aa, synthetic construct
  SOURCE 1..25
PEEEDEEPGDPREGEEEEEEDEPDP

SEQ ID NO: 919 - protein, 25 aa, synthetic construct
  SOURCE 1..25
EEEDEEPGDPREGEEEEEEDEPDPE

SEQ ID NO: 920 - protein, 25 aa, synthetic construct
  SOURCE 1..25
EEDEEPGDPREGEEEEEEDEPDPEA

SEQ ID NO: 921 - protein, 25 aa, synthetic construct
  SOURCE 1..25
EDEEPGDPREGEEEEEEDEPDPEAP

SEQ ID NO: 922 - protein, 25 aa, synthetic construct
  SOURCE 1..25
DEEPGDPREGEEEEEEDEPDPEAPE

SEQ ID NO: 923 - protein, 25 aa, synthetic construct
  SOURCE 1..25
EEPGDPREGEEEEEEDEPDPEAPEN

SEQ ID NO: 924 - protein, 26 aa, synthetic construct
  SOURCE 1..26
AAPEEEDEEPGDPREGEEEEEEDEPD

SEQ ID NO: 925 - protein, 26 aa, synthetic construct
  SOURCE 1..26
APEEEDEEPGDPREGEEEEEEDEPDP

SEQ ID NO: 926 - protein, 26 aa, synthetic construct
  SOURCE 1..26
PEEEDEEPGDPREGEEEEEEDEPDPE

SEQ ID NO: 927 - protein, 26 aa, synthetic construct
  SOURCE 1..26
EEEDEEPGDPREGEEEEEEDEPDPEA

SEQ ID NO: 928 - protein, 26 aa, synthetic construct
  SOURCE 1..26
EEDEEPGDPREGEEEEEEDEPDPEAP

SEQ ID NO: 929 - protein, 26 aa, synthetic construct
  SOURCE 1..26
EDEEPGDPREGEEEEEEDEPDPEAPE

SEQ ID NO: 930 - protein, 26 aa, synthetic construct
  SOURCE 1..26
DEEPGDPREGEEEEEEDEPDPEAPEN

SEQ ID NO: 931 - protein, 27 aa, synthetic construct
  SOURCE 1..27
AAPEEEDEEPGDPREGEEEEEEDEPDP

SEQ ID NO: 932 - protein, 27 aa, synthetic construct
  SOURCE 1..27
APEEEDEEPGDPREGEEEEEEDEPDPE

SEQ ID NO: 933 - protein, 27 aa, synthetic construct
  SOURCE 1..27
PEEEDEEPGDPREGEEEEEEDEPDPEA

SEQ ID NO: 934 - protein, 27 aa, synthetic construct
  SOURCE 1..27
EEEDEEPGDPREGEEEEEEDEPDPEAP

SEQ ID NO: 935 - protein, 27 aa, synthetic construct
  SOURCE 1..27
EEDEEPGDPREGEEEEEEDEPDPEAPE

SEQ ID NO: 936 - protein, 27 aa, synthetic construct
  SOURCE 1..27
EDEEPGDPREGEEEEEEDEPDPEAPEN

SEQ ID NO: 937 - protein, 28 aa, synthetic construct
  SOURCE 1..28
AAPEEEDEEPGDPREGEEEEEEDEPDPE

SEQ ID NO: 938 - protein, 28 aa, synthetic construct
  SOURCE 1..28
APEEEDEEPGDPREGEEEEEEDEPDPEA

SEQ ID NO: 939 - protein, 28 aa, synthetic construct
  SOURCE 1..28
PEEEDEEPGDPREGEEEEEEDEPDPEAP

SEQ ID NO: 940 - protein, 28 aa, synthetic construct
  SOURCE 1..28
EEEDEEPGDPREGEEEEEEDEPDPEAPE

SEQ ID NO: 941 - protein, 28 aa, synthetic construct
  SOURCE 1..28
EEDEEPGDPREGEEEEEEDEPDPEAPEN

SEQ ID NO: 942 - protein, 29 aa, synthetic construct
  SOURCE 1..29
APEEEDEEPGDPREGEEEEEEDEPDPEAP

SEQ ID NO: 943 - protein, 29 aa, synthetic construct
  SOURCE 1..29
PEEEDEEPGDPREGEEEEEEDEPDPEAPE

SEQ ID NO: 944 - protein, 29 aa, synthetic construct
  SOURCE 1..29
EEEDEEPGDPREGEEEEEEDEPDPEAPEN

SEQ ID NO: 945 - protein, 30 aa, synthetic construct
  SOURCE 1..30
APEEEDEEPGDPREGEEEEEEDEPDPEAPE

SEQ ID NO: 946 - protein, 30 aa, synthetic construct
  SOURCE 1..30
PEEEDEEPGDPREGEEEEEEDEPDPEAPEN

SEQ ID NO: 947 - protein, 31 aa, synthetic construct
  SOURCE 1..31
PRGAAAPEEEDEEPGDPREGEEEEEEDEPDP

SEQ ID NO: 948 - protein, 31 aa, synthetic construct
  SOURCE 1..31
RGAAAPEEEDEEPGDPREGEEEEEEDEPDPE

SEQ ID NO: 949 - protein, 31 aa, synthetic construct
  SOURCE 1..31
AAPEEEDEEPGDPREGEEEEEEDEPDPEAPE

SEQ ID NO: 950 - protein, 31 aa, synthetic construct
  SOURCE 1..31
APEEEDEEPGDPREGEEEEEEDEPDPEAPEN

SEQ ID NO: 951 - protein, 31 aa, synthetic construct
  SOURCE 1..31
PEEEDEEPGDPREGEEEEEEDEPDPEAPENG

SEQ ID NO: 952 - protein, 31 aa, synthetic construct
  SOURCE 1..31
EEEDEEPGDPREGEEEEEEDEPDPEAPENGS

SEQ ID NO: 953 - protein, 32 aa, synthetic construct
  SOURCE 1..32
PRGAAAPEEEDEEPGDPREGEEEEEEDEPDPE

SEQ ID NO: 954 - protein, 32 aa, synthetic construct
  SOURCE 1..32
AAPEEEDEEPGDPREGEEEEEEDEPDPEAPEN

SEQ ID NO: 955 - protein, 32 aa, synthetic construct
  SOURCE 1..32
APEEEDEEPGDPREGEEEEEEDEPDPEAPENG

SEQ ID NO: 956 - protein, 32 aa, synthetic construct
  SOURCE 1..32
PEEEDEEPGDPREGEEEEEEDEPDPEAPENGS

SEQ ID NO: 957 - protein, 33 aa, synthetic construct
  SOURCE 1..33
AAPEEEDEEPGDPREGEEEEEEDEPDPEAPENG

SEQ ID NO: 958 - protein, 33 aa, synthetic construct
  SOURCE 1..33
APEEEDEEPGDPREGEEEEEEDEPDPEAPENGS

SEQ ID NO: 959 - protein, 34 aa, synthetic construct
  SOURCE 1..34
AAPEEEDEEPGDPREGEEEEEEDEPDPEAPENGS

SEQ ID NO: 960 - protein, 20 aa, synthetic construct
  SOURCE 1..20
KPPPSEGSDEEEEEEDEEDE

SEQ ID NO: 961 - protein, 20 aa, synthetic construct
  SOURCE 1..20
PPPSEGSDEEEEEEDEEDEE

SEQ ID NO: 962 - protein, 24 aa, synthetic construct
  SOURCE 1..24
PPPSEGSDEEEEEEDEEDEEERKP

SEQ ID NO: 963 - protein, 25 aa, synthetic construct
  SOURCE 1..25
KPPPSEGSDEEEEEEDEEDEEERKP

SEQ ID NO: 964 - protein, 25 aa, synthetic construct
  SOURCE 1..25
PPPSEGSDEEEEEEDEEDEEERKPQ

SEQ ID NO: 965 - protein, 26 aa, synthetic construct
  SOURCE 1..26
KPPPSEGSDEEEEEEDEEDEEERKPQ

SEQ ID NO: 966 - protein, 20 aa, synthetic construct
  SOURCE 1..20
EEEEEEEEEEEEEEEEAPPP

SEQ ID NO: 967 - protein, 20 aa, synthetic construct
  SOURCE 1..20
EEEEEEEEEEEEEEEAPPPP

SEQ ID NO: 968 - protein, 20 aa, synthetic construct
  SOURCE 1..20
EEEEEEEEEEEEEEAPPPPR

SEQ ID NO: 969 - protein, 21 aa, synthetic construct
  SOURCE 1..21
EEEEEEEEEEEEEEEEAPPPP

SEQ ID NO: 970 - protein, 21 aa, synthetic construct
  SOURCE 1..21
EEEEEEEEEEEEEEEAPPPPR

SEQ ID NO: 971 - protein, 22 aa, synthetic construct
  SOURCE 1..22
EEEEEEEEEEEEEEEEEAPPPP

SEQ ID NO: 972 - protein, 22 aa, synthetic construct
  SOURCE 1..22
EEEEEEEEEEEEEEEEAPPPPR

SEQ ID NO: 973 - protein, 23 aa, synthetic construct
  SOURCE 1..23
EEEEEEEEEEEEEEEEEEAPPPP

SEQ ID NO: 974 - protein, 23 aa, synthetic construct
  SOURCE 1..23
EEEEEEEEEEEEEEEEEAPPPPR

SEQ ID NO: 975 - protein, 24 aa, synthetic construct
  SOURCE 1..24
EEEEEEEEEEEEEEEEEEEAPPPP

SEQ ID NO: 976 - protein, 24 aa, synthetic construct
  SOURCE 1..24
EEEEEEEEEEEEEEEEEEAPPPPR

SEQ ID NO: 977 - protein, 25 aa, synthetic construct
  SOURCE 1..25
EEEEEEEEEEEEEEEEEEEEAPPPP

SEQ ID NO: 978 - protein, 25 aa, synthetic construct
  SOURCE 1..25
EEEEEEEEEEEEEEEEEEEAPPPPR

SEQ ID NO: 979 - protein, 26 aa, synthetic construct
  SOURCE 1..26
EEEEEEEEEEEEEEEEEEEEEAPPPP

SEQ ID NO: 980 - protein, 26 aa, synthetic construct
  SOURCE 1..26
EEEEEEEEEEEEEEEEEEEEAPPPPR

SEQ ID NO: 981 - protein, 33 aa, synthetic construct
  SOURCE 1..33
PDDDEEDEEEEEEEEEEEEEEEEEEEEEAPPPP

SEQ ID NO: 982 - protein, 21 aa, synthetic construct
  SOURCE 1..21
EDSEEESQEEEAEGASEPPPP

SEQ ID NO: 983 - protein, 22 aa, synthetic construct
  SOURCE 1..22
QEDSEEESQEEEAEGASEPPPP

SEQ ID NO: 984 - protein, 24 aa, synthetic construct
  SOURCE 1..24
DHQEDSEEESQEEEAEGASEPPPP

SEQ ID NO: 985 - protein, 20 aa, synthetic construct
  SOURCE 1..20
DQSEEEEEEEKHPPKPAKPE

SEQ ID NO: 986 - protein, 21 aa, synthetic construct
  SOURCE 1..21
PAPAHRPPEDEGEENEGEEDE

SEQ ID NO: 987 - protein, 22 aa, synthetic construct
  SOURCE 1..22
PAPAHRPPEDEGEENEGEEDEE

SEQ ID NO: 988 - protein, 20 aa, synthetic construct
  SOURCE 1..20
QENGQREEEEEEKEPEAEPP

SEQ ID NO: 989 - protein, 24 aa, synthetic construct
  SOURCE 1..24
PAEGQENGQREEEEEEKEPEAEPP

SEQ ID NO: 990 - protein, 20 aa, synthetic construct
  SOURCE 1..20
EQEPEPEPEPEPEPEPEPEP

SEQ ID NO: 991 - protein, 20 aa, synthetic construct
  SOURCE 1..20
QEPEPEPEPEPEPEPEPEPE

SEQ ID NO: 992 - protein, 20 aa, synthetic construct
  SOURCE 1..20
EPEPEPEPEPEPEPEPEPEQ

SEQ ID NO: 993 - protein, 21 aa, synthetic construct
  SOURCE 1..21
EQEPEPEPEPEPEPEPEPEPE

SEQ ID NO: 994 - protein, 21 aa, synthetic construct
  SOURCE 1..21
QEPEPEPEPEPEPEPEPEPEQ

SEQ ID NO: 995 - protein, 22 aa, synthetic construct
  SOURCE 1..22
EQEPEPEPEPEPEPEPEPEPEQ

SEQ ID NO: 996 - protein, 20 aa, synthetic construct
  SOURCE 1..20
PEEEEEEEEEEEPASPPERK

SEQ ID NO: 997 - protein, 22 aa, synthetic construct
  SOURCE 1..22
PSPGSPRGQPQDQDDDEDDEED

SEQ ID NO: 998 - protein, 23 aa, synthetic construct
  SOURCE 1..23
PSPGSPRGQPQDQDDDEDDEEDE

SEQ ID NO: 999 - protein, 24 aa, synthetic construct
  SOURCE 1..24
RPSPGSPRGQPQDQDDDEDDEEDE

SEQ ID NO: 1000 - protein, 24 aa, synthetic construct
  SOURCE 1..24
PSPGSPRGQPQDQDDDEDDEEDEA

SEQ ID NO: 1001 - protein, 20 aa, synthetic construct
  SOURCE 1..20
AEDDDEEDEEEEEEEPDPDP

SEQ ID NO: 1002 - protein, 20 aa, synthetic construct
  SOURCE 1..20
EDDDEEDEEEEEEEPDPDPE

SEQ ID NO: 1003 - protein, 20 aa, synthetic construct
  SOURCE 1..20
KQEPPDPEEDKEENKDDSAS

SEQ ID NO: 1004 - protein, 20 aa, synthetic construct
  SOURCE 1..20
QEPPDPEEDKEENKDDSASK

SEQ ID NO: 1005 - protein, 20 aa, synthetic construct
  SOURCE 1..20
EDEDEDESSEEDSEDEEPPP

SEQ ID NO: 1006 - protein, 20 aa, synthetic construct
  SOURCE 1..20
DEDEDESSEEDSEDEEPPPK

SEQ ID NO: 1007 - protein, 20 aa, synthetic construct
  SOURCE 1..20
EDEDESSEEDSEDEEPPPKR

SEQ ID NO: 1008 - protein, 20 aa, synthetic construct
  SOURCE 1..20
DEDESSEEDSEDEEPPPKRR

SEQ ID NO: 1009 - protein, 26 aa, synthetic construct
  SOURCE 1..26
PDDSRDEDEDEDESSEEDSEDEEPPP

SEQ ID NO: 1010 - protein, 30 aa, synthetic construct
  SOURCE 1..30
PKKEPDDSRDEDEDEDESSEEDSEDEEPPP

SEQ ID NO: 1011 - protein, 31 aa, synthetic construct
  SOURCE 1..31
PKKEPDDSRDEDEDEDESSEEDSEDEEPPPK

SEQ ID NO: 1012 - protein, 32 aa, synthetic construct
  SOURCE 1..32
PKKEPDDSRDEDEDEDESSEEDSEDEEPPPKR

SEQ ID NO: 1013 - protein, 33 aa, synthetic construct
  SOURCE 1..33
PKKEPDDSRDEDEDEDESSEEDSEDEEPPPKRR

SEQ ID NO: 1014 - protein, 21 aa, synthetic construct
  SOURCE 1..21
PEEEAAEEEEEEEERPKPSRP

SEQ ID NO: 1015 - protein, 22 aa, synthetic construct
  SOURCE 1..22
QPEEEAAEEEEEEEERPKPSRP

SEQ ID NO: 1016 - protein, 23 aa, synthetic construct
  SOURCE 1..23
EQPEEEAAEEEEEEEERPKPSRP

SEQ ID NO: 1017 - protein, 24 aa, synthetic construct
  SOURCE 1..24
EEQPEEEAAEEEEEEEERPKPSRP

SEQ ID NO: 1018 - protein, 25 aa, synthetic construct
  SOURCE 1..25
EEEQPEEEAAEEEEEEEERPKPSRP

SEQ ID NO: 1019 - protein, 22 aa, synthetic construct
  SOURCE 1..22
PEEEDDEAQQPQPQSGPEEAEE

SEQ ID NO: 1020 - protein, 24 aa, synthetic construct
  SOURCE 1..24
DKPEEEDDEAQQPQPQSGPEEAEE

SEQ ID NO: 1021 - protein, 24 aa, synthetic construct
  SOURCE 1..24
PEEEDDEAQQPQPQSGPEEAEEGE

SEQ ID NO: 1022 - protein, 25 aa, synthetic construct
  SOURCE 1..25
PEEEDDEAQQPQPQSGPEEAEEGEE

SEQ ID NO: 1023 - protein, 26 aa, synthetic construct
  SOURCE 1..26
EGDKPEEEDDEAQQPQPQSGPEEAEE

SEQ ID NO: 1024 - protein, 26 aa, synthetic construct
  SOURCE 1..26
DKPEEEDDEAQQPQPQSGPEEAEEGE

SEQ ID NO: 1025 - protein, 26 aa, synthetic construct
  SOURCE 1..26
KPEEEDDEAQQPQPQSGPEEAEEGEE

SEQ ID NO: 1026 - protein, 26 aa, synthetic construct
  SOURCE 1..26
PEEEDDEAQQPQPQSGPEEAEEGEEE

SEQ ID NO: 1027 - protein, 32 aa, synthetic construct
  SOURCE 1..32
PEEEDDEAQQPQPQSGPEEAEEGEEEEAERGP

SEQ ID NO: 1028 - protein, 33 aa, synthetic construct
  SOURCE 1..33
KPEEEDDEAQQPQPQSGPEEAEEGEEEEAERGP

SEQ ID NO: 1029 - protein, 20 aa, synthetic construct
  SOURCE 1..20
NNSEEEEDDDDEEEEPDKPP

SEQ ID NO: 1030 - protein, 20 aa, synthetic construct
  SOURCE 1..20
NSEEEEDDDDEEEEPDKPPA

SEQ ID NO: 1031 - protein, 20 aa, synthetic construct
  SOURCE 1..20
SEEEEDDDDEEEEPDKPPAN

SEQ ID NO: 1032 - protein, 125 aa, synthetic construct
  SOURCE 1..125
QVQLQQSGGGLVQPGGSLRLSCAASGFTLDYYAIGWFRQAPGKEREGVLCISSSGGSTNYADSVKGRFTISRDNAKNTVYLQMNSLKPEDTAVYYCAADDLRCGSNWSSYFRGSWGQGTQVTVSS

SEQ ID NO: 1033 - protein, 241 aa, synthetic construct
  SOURCE 1..241
AEVQLLESGGGLVQPGGSLRLSCAASGFTFSSYAMSWVRQAPGKGLEWVSYIASGGDTTNYADSVKGRFTISRDNSKNTLYLQMNSLRAEDTAVYYCAKGASAFDYWGQGTLVTVSSGGGGSGGGGSGGGGSTDIQMTQSPSSLSASVGDRVTITCRASQSISSYLNWYQQKPGKAPKLLIYAASYLQSGVPSRFSGSGSGTDFTLTISSLQPEDFATYYCQQSSNDPYTFGQGTKVEIKR

SEQ ID NO: 1034 - protein, 22 aa, synthetic construct
  SOURCE 1..22
MARVKKDQAEPLHRKFERQPPG

SEQ ID NO: 1035 - protein, 242 aa, synthetic construct
  SOURCE 1..242
EVQLLESGGGLVQPGGSLRLSCAASGFTFSSYAMSWVRQAPGKGLEWVSAISGSGGSTYYADSVKGRFTISRDNSKNTLYLQMNSLRAEDTAVYYCAKMRLGLFDYWGQGTLVTVSSGGGGSGGGGSGGGGEIVLTQSPGTLSLSPGERATLSCRASQSVSSSYLAWYQQKPGQAPRLLIYGASSRATGIPDRFSGSGSGTDFTLTISRLEPEDFAVYYCQQRGDVPPTFGQGTKVEIKAAA

SEQ ID NO: 1036 - protein, 49 aa, synthetic construct
  SOURCE 1..49
YPYDVPDYAGSPQPVEDGEDEFCTPMACEANIQSGDSAAPMSAVHRHRL

SEQ ID NO: 1037 - protein, 49 aa, synthetic construct
  SOURCE 1..49
NNYDVPDNAGSPQPQEDGEDEFNNPQANEANQQSGDSNNPNSAVNRHNN

SEQ ID NO: 1038 - protein, 50 aa, synthetic construct
  SOURCE 1..50
MTRGNQRELARQKNMKKQSDSVKGKRRDDGLSAAARKQRDSEIMQQKQKK

SEQ ID NO: 1039 - protein, 83 aa, synthetic construct
  SOURCE 1..83
MSGPNGDLGMPVEAGAEGEEDGFGEAEYAAINSMLDQINSCLDHLEEKNDHLHARLQELLESNRQTRLEFQQQLGEAPSDASP

SEQ ID NO: 1040 - protein, 99 aa, synthetic construct
  SOURCE 1..99
MAQGQRKFQAHKPAKSKTAAAASEKNRGPRKGGRVIAPKKARVVQQQKLKKNLEVGIRKKIEHDVVMKASSSLPKKLALLKAPAKKKGAAAATSSKTPS

SEQ ID NO: 1041 - protein, 35 aa, synthetic construct
  SOURCE 1..35
NDEYSDFEDSDFDGDYKDSDEDYKDDSENFDDGFE

SEQ ID NO: 1042 - protein, 35 aa, synthetic construct
  SOURCE 1..35
PDEPPDPEDPDPDPDPKDPDEDPKDDPEPPDDPPE

SEQ ID NO: 1043 - protein, 35 aa, synthetic construct
  SOURCE 1..35
NDEPPDPEDSDPDGDPKDSDEDPKDDSEPPDDGPE